European Patent Specification EP 3 552 126 B1, published May 14, 2025. Title: SYSTEMS AND METHODS FOR SEQUENCING T CELL RECEPTORS AND USES THEREOF. Applicant: Regeneron Pharmaceuticals, Inc. The sequence listing filed with the application follows.

SEQUENCE LISTING (324 sequences)

SEQ ID NO: 1 - protein, 121 aa, Artificial Sequence
  synthetic construct; antigen binding domain
EVQLLESGGGLVQPGGSLRLSCSASGFTFSSYTMNWVRQAPGKGLEWVSGISDTGGNTYYTDSVKGRFTVSRDNSKNTLSLQMNSLRAEDTAVYYCAKDQGGSYPYYFHYWGQGSLVTVSS

SEQ ID NO: 2 - protein, 108 aa, Artificial Sequence
  synthetic construct; antigen binding domain
DIQMTQSPSSLSASVGDRVTITCRASQSISSYLIWYQQKPGTAPKFLIYAASSLQSGVPSRFSGCGSGTDFTLTISSLQPEDFATYYCQQSYSTPPITFGQGTRLEIK

SEQ ID NO: 3 - protein, 122 aa, Artificial Sequence
  synthetic construct; antigen binding domain
EVQLVESGGGLVQPGGSLRLSCAASGFTVSNNYMSWVRQAPGKGLEWVSVIYSGGFTYYTDSVKGRFTISRHNSKNTLYLQMNSLRAEDTAVYYCARYYYDTSDYWTFFDYWGQGTLVTVSS

SEQ ID NO: 4 - protein, 107 aa, Artificial Sequence
  synthetic construct; antigen binding domain
EIVMTQSPATLSVSPGERATLSCRASQSVSSNLAWYQQKPGQAPRLLIYGASTRATGIPARFSGSGSGTEFTLTISSLQSGDFAVYYCQQYNNWPLTFGGGTKVEIN

SEQ ID NO: 5 - protein, 122 aa, Artificial Sequence; identical to SEQ ID NO: 3
  synthetic construct; antigen binding domain

SEQ ID NO: 6 - protein, 107 aa, Artificial Sequence; identical to SEQ ID NO: 4
  synthetic construct; antigen binding domain

SEQ ID NO: 7 - protein, 119 aa, Artificial Sequence
  synthetic construct; antigen binding domain
QVQLVESGGGVVQSGRSLRLSCAASGFTFSSYGMHWVRQAPGKGLEWVAVIWYDGSNIYYSDSVKGRFTISRANSKNTLYLQMNSLRAEDTAVYYCARPGHWNYFFEYWGQGTLVTVSS

SEQ ID NO: 8 - protein, 108 aa, Artificial Sequence
  synthetic construct; antigen binding domain
DIQMTQSPSSLSASVGDRVTITCRASQSINNYLNWYQQKPGKAPKLLIYTASSLQSGVPSRFSGSGSGTDFTLTISSLQPEDFATYYCQQSYSTPPLTFGQGTQLEIK

SEQ ID NO: 9 - protein, 122 aa, Artificial Sequence
  synthetic construct; antigen binding domain
EVQLVESGGGLVQPGGSLRLSCGASGFTFRNYDMHWVRQITGKGLEWVSAIGSAGDTYYPDSVKGRFTISRENAKNSLYLQMNSLRVGDTAVYYCTRDIHCSSTRCYGMDVWGQGTTVTVSS

SEQ ID NO: 10 - protein, 108 aa, Artificial Sequence
  synthetic construct; antigen binding domain
DIQMTQSPSSLSASVGDRVTITCRASQSISNYLNWYQQKPGKAPKLLIYAASSLQSGVPSRFSGSGSGTDFTLTISSLQPEDFATYYCQQSYSTPPITFGQGTRLEIK

SEQ ID NO: 11 - protein, 130 aa, Artificial Sequence
  synthetic construct; antigen binding domain
EVQLVESGGGLVKPGGSLRLSCAASGFKFSNEWMSWVRQAPGKGLEWVGRIKSKTDGGTTDYAAPVKGRFTISRDDSKNTLYLQMNSLKTEDTAVYYCTTDQDFWSGYYTGADYYGMDVWGQGTMVTVSS

SEQ ID NO: 12 - protein, 108 aa, Artificial Sequence
  synthetic construct; antigen binding domain
DIQMTQSPSSLSASVGDRVTITCRASQSISSYLNWYQQKPGKAPKLLIYAASSLQSGVPSRFSGSGSGTDFTLTISSLQPEDFATYYCQQSYSTPPITFGQGTRLEIK

SEQ ID NO: 13 - protein, 116 aa, Artificial Sequence
  synthetic construct; antigen binding domain
QMQLQQWGAGLLKPSETLSLTCVVYGGSLNGYYWSWIRQSPGKGLEWIGEIDHSGSTNYNPSLKNRVTMSVDTSKIQFSLKLTSVTVADTAVYYCAREGLLPFDYWGQGTLVTVSS

SEQ ID NO: 14 - protein, 108 aa, Artificial Sequence
  synthetic construct; antigen binding domain
EIVLTQSPGTLSLSPGERVTLSCRASQSVYSNYLAWYQQNPGQAPRLLIYAASNRATGIPDRFSGSGSGTDFTLTISRLEPEDFAVYYCHQYATSPWTFGQGTKVEIK

SEQ ID NO: 15 - protein, 123 aa, Artificial Sequence
  synthetic construct; antigen binding domain
QLQLQESGPDLVKPSDTLSLTCTVSDDSISSTTYYWAWIRQPPGKGLEWIGSMSYNGNNYYNPSLKSRVAISAGTSQKQFSLKLTSVTAADTAVYHCARHLGYNGNWYPFDFWGQGILVTVSS

SEQ ID NO: 16 - protein, 108 aa, Artificial Sequence
  synthetic construct; antigen binding domain
EIVLTQSPGTLSLSPGERATLSCRASQSVSSSYLAWYQQKPGQAPRLLIYGASSRTTGIPDRFSGSGSGTDFTLTISRLEPEDFAVYYCQQYGSSPWTFGQGTKVEIK

SEQ ID NO: 17 - protein, 122 aa, Artificial Sequence
  synthetic construct; antigen binding domain
EVQVVESGGGLVEPGRSLRLSCKASGFTFDDYAMHWVRQTPGKALEWVSGINWSGNNIGYADSVKGRFTISKDDAKNSLYLQMNSLRPEDTALYYCTKDISITGTLDAFDVWGQGTMVTVSS

SEQ ID NO: 18 - protein, 107 aa, Artificial Sequence
  synthetic construct; antigen binding domain
DIQMTQSPISVSASVGDRVTITCRASQGISNWLAWYQQKPGIAPKLLIYSASSLQSGVPSRFRGSGSGTDFTLTIGSLQPEDFATYYCQQAHSFPLTFGGGTKVEIK

SEQ ID NO: 19 - protein, 116 aa, Artificial Sequence
  synthetic construct; antigen binding domain
QVQLVESGGGVVQPGRSLRLSCAASGFTFSSYGMHWVRQAPGKGLEWVAIIWSDGDSEYNLDSVKGRFTISRDNSKNTLYLQMNSLRVEDSAVYYCARDRDLEDIWGQGTMVTVSS

SEQ ID NO: 20 - protein, 107 aa, Artificial Sequence
  synthetic construct; antigen binding domain
DIQMTQSPSSLSASVGDRVTITCRASQGIRNDLGWYQQKPGKAPKRLIYAASNLQSGVPSRFSGSGSGTEFTLTISSLQPEDFATYYCLQHNSYPLTFGGGTKVEIK

SEQ ID NO: 21 - protein, 117 aa, Artificial Sequence [sequence omitted]

SEQ ID NO: 22 - protein, 107 aa, Artificial Sequence [sequence omitted]

SEQ ID NO: 23 - protein, 121 aa, Artificial Sequence
  synthetic construct; antigen binding domain
EVQLVESGGGVVRPGGSLRLSCAASGFTFDDYGMSWVRQVPGKGLEWVSGISWNDGKTVYAESVKGRFIISRDNAKNSLYLEMNSLRAEDTALYYCARDWQYLIERYFDYWGQGTLVTVSS

SEQ ID NO: 24 - protein, 108 aa, Artificial Sequence
  synthetic construct; antigen binding domain
EIVLTQSPGTLSLSPGERATLSCRASQSVSSSYLAWYQQKPGQAPRLLIYGASSRATGIPDRFSGSGSGTDFTLTISRLEPEDFAVYYCQQYGSSPWTFGQGTKVEIK

SEQ ID NO: 25 - protein, 121 aa, Artificial Sequence
  synthetic construct; antigen binding domain
EVQLVESGGGVVRPGGSLRLSCTASGFTFDDYGMSWVRQAPGKGLEWISGIGWTGGRSSYADSVRGRFTISRDNAKNSLYLQMNSLGAEDTALYYCARDRQWLVQWYFDYWGQGTLVTVSS

SEQ ID NO: 26 - protein, 108 aa, Artificial Sequence; identical to SEQ ID NO: 12
  synthetic construct; antigen binding domain

SEQ ID NO: 27 - protein, 121 aa, Artificial Sequence
  synthetic construct; antigen binding domain
EVQLVESGGRVVRPGGSLRLSCAASGFTFDDYGMSWVRQLPGKGLEWVAGISWNDGKTVYAESVKGRFIISRDNAKNSLHLEMNSLRAEDTALYYCARDWQYLIDRYFDFWGQGTLVTVSS

SEQ ID NO: 28 - protein, 121 aa, Artificial Sequence
  synthetic construct; antigen binding domain
EVQLVESGGGLVQPGGSLRLSCAASGFTFDDYAMHWVRQAPGKGLEWVSGIGWSSGSIGYADSVKGRFTISRDNAKNSLYLQMDSLRPEDSALYYCAKAYTFMITLYFDYWGQGTLVTVSS

SEQ ID NO: 29 - protein, 121 aa, Artificial Sequence
  synthetic construct; antigen binding domain
EVQLVESGGGLVQPGRSLRLSCAASGFTFDDYDMHWVRQAPGKGLEWVSGSGWNRGSLGYADSVKGRFTISRDNAKKSLYLQMNSVRVEDTALYYCAKGFVVVSAAYFDYWGQGTLVTVSS

SEQ ID NO: 30 - protein, 121 aa, Artificial Sequence
  synthetic construct; antigen binding domain
QVQLVQSGAEVKRPGSSVKVSCKVSGVTFRNFAIIWVRQAPGQGLEWMGGIIPFFSAANYAQSFQGRVTITPDESTSTAFMELASLRSEDTAVYYCAREGERGHTYGFDYWGQGTLVTVSS

SEQ ID NO: 31 - protein, 121 aa, Artificial Sequence
  synthetic construct; antigen binding domain
EVQLVESGGGLVQSGRSLRLSCAASGFTFDDYAMHWVRQPPGKGLEWVSGINWNRGRTGYADSVKGRFTISRDNAKNSLYLQMNDLRVEDTALYYCAKAEQWLDEGYFDYWGQGTLVTVSS

SEQ ID NO: 32 - protein, 121 aa, Artificial Sequence
  synthetic construct; antigen binding domain
EVQLVESGGGLVQRGGSLRLSCAASGFSFSSYAMNWVRQAPGKGLEWVSTISDSGGSTYYADSVKGRFTISRDNSKNTLSLQMNSLRAEDTAVYYCAKDQGGSYPYYFHYWGQGTLVTVSS

SEQ ID NO: 33 - protein, 121 aa, Artificial Sequence
  synthetic construct; antigen binding domain
EVQLVESGGGLVQPGRSLRLSCAASGFTFEDYAMHWVRQAPGKGLEWVSGIGWSNVKIGYADSVKGRFTISRDNVRNSLYLQMNSLRTEDTAFYYCVKAYTSMLTLYFDYWGQGTLVTVSS

SEQ ID NO: 34 - protein, 118 aa, Artificial Sequence
  synthetic construct; antigen binding domain
QVQLVQSGAEVKRPGASVKVSCKASGYTFTSFYMYWVRQAPGQGLEWMGIINPSDGSTSNAQKFQGRVTMTRDTSTSTVYMELSSLRSEDTAVYYCARRVAGDIFDIWGQGTMVTVSS

SEQ ID NO: 35 - protein, 119 aa, Artificial Sequence
  synthetic construct; antigen binding domain
QVQLQESGPGLVKPSETLSLTCTVSGGSISSYHWNWIRQSPGKGLEWIGYIYYIGSTDYNPSLESRVTISVDTSKNQFSLKLSSVTAADTAVYYCARVPVGATGASDVWGQGTMVTVSS

SEQ ID NO: 36 - protein, 121 aa, Artificial Sequence
  synthetic construct; antigen binding domain
EVQLVESGGSVVRPGGSLRLSCVVSGFTFEDYGLSWVRQIPGKGLEWVSGISWTGGNTGYADSVKGRFTISRDNAKNSLYLQMNSLRAEDTALYHCTRDRQWLMQWYFDYWGQGTLVTVSS

SEQ ID NO: 37 - protein, 119 aa, Artificial Sequence
  synthetic construct; antigen binding domain
QVQLVESGGGVVQPGRSLRLSCSASGFTFSAYAMHWVRQAPGKGLEWVAAISYGGSDKYYADSVKGRFTISRDNSKNTLYLQMNSLRTDDTAVYYCAKSAHWNFFFDYWGQGTLVTVSS

SEQ ID NO: 38 - protein, 121 aa, Artificial Sequence
  synthetic construct; antigen binding domain
EVQLVESGGGLVQPGRSLRLSCVASGFALHDYAMHWVRQVPGKGLEWVSSISWNSGVIGYADSLKGRFTISRDNAKNSLYLQMNSLRAEDTALYYCAKGSGSYYVSWFDPWGQGTLVTVSS

SEQ ID NO: 39 - protein, 123 aa, Artificial Sequence
  synthetic construct; antigen binding domain
QLQLQESGPGLVQPSETLSLTCTVSGDSISSTAYHWDWIRQPPGKGLEWIGTITYNGNTYFNPSLKSRVTISVDTSKNQFSLKLLSMTAAETAVFYCARHLGYNSDFFPFDFWGQGTLVTVSS

SEQ ID NO: 40 - protein, 119 aa, Artificial Sequence
  synthetic construct; antigen binding domain
EVQLVESGGGLVRPGGSLRLSCAASGFTFSTYAMAWVRQTPGKGLEGVSAIGGSGDSTYYVDSVKGRFTISRDNSKSTLFLQMNSLRAEDTAVYYCVKVRNYDGSFDIWGQGTMVTVSS

SEQ ID NO: 41 - protein, 124 aa, Artificial Sequence
  synthetic construct; antigen binding domain
EVQLLESGGGLVQPGGSLRLSCVASGFTFSTYAMSWVRQAPGMGLEWVSSISGSGRNTYYADSVKGRFTISRDNSKNTLFLQMNSLRAEDTAVYYCAKESVTGTSSYYYGVDVWGQGTTVTVSS

SEQ ID NO: 42 - protein, 107 aa, Artificial Sequence
  synthetic construct; antigen binding domain
DIQMTQSPSSLSASVGDRVTITCRASQSISSYLNWYHQKPGKAPKLLIYAASSLQNGVPSRFSGSGSGTDFTLTISSLQPEDFASYYCQQSYRTPLTFGGGTKVEIK

SEQ ID NO: 43 - protein, 128 aa, Artificial Sequence
  synthetic construct; antigen binding domain
QVQLEESGGGVVQPGRSLRLSCAASGFTFSWYGMHWVRQAPGKGLEWVALIWYDGTNKKYGDSVKGRFTISRDNSKNTVYLQMNSLRAEDTAVYYCARDCGHSGNDRGTYYYYYGMDVWGQGTTVTVS

SEQ ID NO: 44 - protein, 108 aa, Artificial Sequence; identical to SEQ ID NO: 12
  synthetic construct; antigen binding domain

SEQ ID NO: 45 - protein, 119 aa, Artificial Sequence
  synthetic construct; antigen binding domain
QVQLQQWGAGLLKPSETLSLTCAVYGGSFSGYYWNWIRQPPGKGLEWVGEISHRGTTNYNPSLKSRVTISLDTSKNQFSLKLTSVTAADTAVYYCSRDEELEFRFFDYWGQGTLVTVSS

SEQ ID NO: 46 - protein, 107 aa, Artificial Sequence
  synthetic construct; antigen binding domain
EIVLTQSPATLSLSPGERATLSCRASQSVSSYLAWYQQKPGQAPRLLVYGASNRATGIPARFSGSGSGTDFTLTISSLEPEDFAFYYCQQRSNWPLTFGGGTKVEIK

SEQ ID NO: 47 - protein, 119 aa, Artificial Sequence
  synthetic construct; antigen binding domain
QLQLQESGPGLVKPSETLSLTCTVSGDSIISNSYYWGWIRQPPGKGLEWIGNFFYTGATYYNPSLKSRVTISADTSKNQFSLKLSSVTAADTALYYCASYNRNYRFDPWGQGTLVTVSS

SEQ ID NO: 48 - protein, 108 aa, Artificial Sequence
  synthetic construct; antigen binding domain
DIQMTQSPSSLSASVGDRVTITCRASQSISSYLNWYQQKPGKAPKLLIYAASSLQSGVPSRFSGSGSGTDFTLTISSLQPEDFATYFCQQSYSTPPITFGQGTRLEIK

SEQ ID NO: 49 - protein, 127 aa, Artificial Sequence
  synthetic construct; antigen binding domain
QVQLQQWGAGLLKPSETLSLTCAVYGGSFSTYYWSWIRQPPGKGLEWIGEINHSGNADYNPSLKSRVSISVDTSKNQFSLRLSSVTAADTAIYYCARAGYCSSPTCYSYYYFGMDVWGQGTTVTVSS

SEQ ID NO: 50 - protein, 108 aa, Artificial Sequence
  synthetic construct; antigen binding domain
EIVLTQSPGTLSLSLGERATLSCRASQSVISSFLAWYQQKPGQAPRLLIYGASSRATGFPDRFSGSGSGTDFTLTIRRLEPEDFAVYYCQQYGNSPWTFGQGTKVEIK

SEQ ID NO: 51 - protein, 129 aa, Artificial Sequence
  synthetic construct; antigen binding domain
QVTLKESGPVLVKPTETLTLTCTVSGFSLSNAGMGVSWVRQPPGKALEWLAHIFSNDEKSYSTSLRTRLTISKDTSKSQVVLTVTNLDPVDTATYFCARIPEFTSSSWALYYFYGMDVWGQGTTVTVSS

SEQ ID NO: 52 - protein, 108 aa, Artificial Sequence
  synthetic construct; antigen binding domain
EIVLTQSPGTLSLSPGESATLSCRASQSITSTYFAWYQQKPGQAPRLLIYATSSRATGVPDRFSGSGSGTDFTLTISRLEPDDFAVYYCQQYGRSPWTFGQGTKVEVK

SEQ ID NO: 53 - protein, 121 aa, Artificial Sequence
  synthetic construct; antigen binding domain
QVQLVQSGAEVKKPGASVKVSCKASGYTFTSYGISWVRQAPGQGLEWMGWISAYNDNTNYAQKLQGRVTMTADTSTNTAYMELRSLRSDDTAIYYCVRWNWGSVYWYFDLWGRGTLVTVSS

SEQ ID NO: 54 - protein, 108 aa, Artificial Sequence
  synthetic construct; antigen binding domain
EIVLTQSPGTLSLSPGERATLSCRASQIISSSYFAWYQQKPGQAPRLLIYGASSRATGIPDRFSGSVSGTDFTLTISRLEPEDFAMYFCQQYGNSPWTFGQGTKVEIK

SEQ ID NO: 55 - protein, 117 aa, Artificial Sequence
  synthetic construct; antigen binding domain
QITLKESGPTLVKPTQTLTLTCTFSGFSLNTHRVGVGWIRQPPGKALEWLALIYGNDVKNYSPSLETRLTIAKDTSKNQVVLTMTNMDPVDTATYFCSYITGEGMYWGQGTLVTVSS

SEQ ID NO: 56 - protein, 111 aa, Artificial Sequence
  synthetic construct; antigen binding domain
DVVMTQSPLSLSVTLGQPASISCRSSQNLMYSDGNTYLNWFHQRPGQSPRRLIYKVSNRDSGVPDRFSGSGSGTDFTLKISRVEAEDVGVYYCMQGTHWYTFGQGTKLEIK

SEQ ID NO: 57 - protein, 119 aa, Artificial Sequence
  synthetic construct; antigen binding domain
QVQLQQWGAGLLKPSETLSLTCAVYGGSFSGYYWSWIRQPPGKGLEWIGEINHRGNTNYNPSLKSRVTISLDTSKKQFSLNLSSVTAADTAMYYCTRDEEQELRFLDYWGQGTLVTVSS

SEQ ID NO: 58 - protein, 107 aa, Artificial Sequence
  synthetic construct; antigen binding domain
EIVLTQSPATLSLSPGERATLSCRASQDISTYLAWYQQRAGQAPRLLIYGASNRATGIPARFSGSGSGTDFTLTISSLEPEDFAFYYCQQRSNWPLTFGGGTEVEIK

SEQ ID NO: 59 - protein, 122 aa, Artificial Sequence
  synthetic construct; antigen binding domain
QVQLQQWGAGLLKPSETLSLTCVVHGGSFSGYYWNWIRQPPGKGLEWIGEINHRGNTNYNPSLKSRVTVSEDTSKNQFSLKLSSLTAADTAVYYCVRGEDYDFWSDYYNDYWGQGTLVTVSS

SEQ ID NO: 60 - protein, 107 aa, Artificial Sequence
  synthetic construct; antigen binding domain
EIVLTQSPATLSLSPGERATLSCRASQTISSYLAWHQQKPGQAPRLLIYDASKRATGIPARFSGSGSGTDFTLTITSLEPEDFAVYYCQQRSNWPLTFGGGTKVEIK

SEQ ID NO: 61 - protein, 124 aa, Artificial Sequence
  synthetic construct; antigen binding domain
QVQLQQWGAGLLPPSETLSLICAVYGGSFSGYYWSWIRQPPGKGLEWIGEINHRGSTNYNPSLKSRATISVDTSKNQFSLKLSSVTAADTAVYYCSRGEDYYDSSGYSYYFDYWGQGTLVTVSS

SEQ ID NO: 62 - protein, 107 aa, Artificial Sequence
  synthetic construct; antigen binding domain
EIVLTQSPATLSLSPGERATLSCRASQSVSSYLAWYQQKPGQAPRLLIYDASNRATGIPARFSGSGSGTDFTLTISSLEPEDFAVYYCQQRSNWPLTFGGGTKVEIK

SEQ ID NO: 63 - protein, 122 aa, Artificial Sequence
  synthetic construct; antigen binding domain
QVQLQQWGAGLLRPSETLSLTCAVYGGSFSGYYWNWIRQSPGTGLEWIGEINHRGNINFNPSLKSRVTISEDTSKNQFSLRLNSVTAADTAVYYCARGEDYDIWSGYYREYWGQGTLVTVSS

SEQ ID NO: 64 - protein, 107 aa, Artificial Sequence
  synthetic construct; antigen binding domain
EIVLTQSPATLSLSPGERATLSCRASQSVSSYLAWYQQKPGQAPRLLIYDASKRATGIPARFSGSGSGTDFTLTISSLEPEDFAVYYCQQRSNWPLAFGGGTKVEIK

SEQ ID NO: 65 - protein, 119 aa, Artificial Sequence
  synthetic construct; antigen binding domain
QVQLQQWGAGLLKPSETLSLTCAVYGGSFSEFYWNWIRQPPEKGLEWIGEINHRGNTNYNPSLKSRVTISVDMSKNQFSLQLNSVTVADTALYYCAFGYDFRSSYEDVWGQGTTVTVSS

SEQ ID NO: 66 - protein, 107 aa, Artificial Sequence
  synthetic construct; antigen binding domain
EIVLTQSPATLSLSPGERATLSCRASQDISTYLAWHQQKPGQPPRLLIYGSSNRATGIPARFSGSGSGTDFTLTISSLEPEDFAVYYCQQRSNWPLTFGGGTKVEIK

SEQ ID NO: 67 - protein, 124 aa, Artificial Sequence
  synthetic construct; antigen binding domain
EVQLLESGGGLVQPGGSLRLSCAASGFTFRSYAMSWVRQAPGKGLEWVSVISGGGGRTYYTDSVKGRFTISRDNSKSMLYLQMNSLRAEDTAIYYCAKERVTGIDHYYYGVDVWGQGTTVTVSS

SEQ ID NO: 68 - protein, 107 aa, Artificial Sequence
  synthetic construct; antigen binding domain
DIQMTQSPSSLSASVGDRVTITCRASQSISSYLNWYQQKPGKAPKLLIYATSSLQSGVPSRFSGSASGTDFTLAISSLQPEDFATYYCQQSYTTPLTFGGGTKVEIK

SEQ ID NO: 69 - protein, 130 aa, Artificial Sequence
  synthetic construct; antigen binding domain
EVQLVESGGGLVQPGGSLRLSCAASGFTFSSYEMNWVRQAPGKGLEWVSYISSSGNTKDYAGSVKGRVTISRDNAKNLLYLQMNSLRAEDTAVYHCARDGGHYDILTGSMSYYYYALDVWGQGTTVTVSS

SEQ ID NO: 70 - protein, 108 aa, Artificial Sequence; identical to SEQ ID NO: 12
  synthetic construct; antigen binding domain

SEQ ID NO: 71 - protein, 121 aa, Artificial Sequence
  synthetic construct; antigen binding domain
EVQLVESGGGLVQPGGSLRLSCAASGFTFKTYAMSWVRQAPGRGLEWVSGISGSGSTSYYADSVKGRFTISRDNYKKTLSLQMNSLRAEDTAVYYCALDIMATVGGLFNNWGQGTLVTVSS

SEQ ID NO: 72 - protein, 108 aa, Artificial Sequence; identical to SEQ ID NO: 24
  synthetic construct; antigen binding domain

SEQ ID NO: 73 - protein, 120 aa, Artificial Sequence
  synthetic construct; antigen binding domain
QVQLVQSGAEVKKPGSSVKVSCKASGGTFSRHTISWVRQAPGQGLEWMGGIIPIFGTANYAHKFQGRVTITTDESTSTAYMELSSLRSEDTAVYYCARAPYTRQGYFDLWGRGTLVTVSS

SEQ ID NO: 74 - protein, 113 aa, Artificial Sequence
  synthetic construct; antigen binding domain
DIVMTQSPDSLAVSLGERATINCKSSQSVLYSSNNKNYLAWYQQKPGQPPKLLIYWASTRESGVPDRFSGSGSGTDFTLTISSLQAEDVAVYYCQQDYSTPWTFGQGTKVEIK

SEQ ID NO: 75 - protein, 118 aa, Artificial Sequence
  synthetic construct; antigen binding domain
QVQLVQSGAEVKKPGASVKVSCKASGYTFTNYYIHWVRQAPGQGLDWMGIINPGGGNTNYAQKFLGRVTMTRDTSTTTVYMELSSLRSEDTAIYYCARENWNSYFDNWGQGTLVTVSS

SEQ ID NO: 76 - protein, 113 aa, Artificial Sequence
  synthetic construct; antigen binding domain
DIVMTQSPDSLAVSLGERATINCKSSQSVLYSSNNKNFLAWYQQKPGQPPKLLIYWASTRESGVPDRFSGSGSGTDFTLTISSLQAEDVALYYCQQYYGAPWTFGQGTKVEIK

SEQ ID NO: 77 - protein, 119 aa, Artificial Sequence
  synthetic construct; antigen binding domain
QVQLVQSGAEVKKPGSSVKVSCKASGGTFSSYTINWVRQAPGQGLEWMGGIIPIFGIANYAQKFQGRVTITTDESTNTAYMELSSLRSEDTAIYYCARARYGSGSYDYWGQGTLVTVSS

SEQ ID NO: 78 - protein, 113 aa, Artificial Sequence
  synthetic construct; antigen binding domain
DIVMTQSPDSLAVSLGERATINCKSSQSVLYTSNNKNYLAWYQQKPGQPPKLLIYWASTRESGVPDRFSGSGSGTDFTLTISSLQAEDVAVYYCQQYYNTPWTFGQGTKVEIK

SEQ ID NO: 79 - protein, 120 aa, Artificial Sequence
  synthetic construct; antigen binding domain
QITLKESGPTLVKPTQTLTLTCTFSGFSLSTNGVGVGWIRQPPGKALEWLGIIYWNDDKRYSPSLRSRLTITKDTSKNQVVLTMTNMDPVDTATYYCAHRGLFGGWFDPWGQGTLVTVSS

SEQ ID NO: 80 - protein, 107 aa, Artificial Sequence
  synthetic construct; antigen binding domain
DIQMTQSPSSLSASVGDRVTITCRASQSISRYLNWYQQKPGKAPNLLIFAASSLQSGVPSRFSGSGSGTDFTLTISSLQPEDFATYFCQQSYNTPLTFGGGTKVEIK

SEQ ID NO: 81 - protein, 122 aa, Artificial Sequence
  synthetic construct; antigen binding domain
EVQLVESGGGLVQPGGSLRLSCAISGFTFRSYAMTWVRQAPGKALEWVSVISGSGGNTYYADSVKGRFTVSRDNSRNTLYLQMNSLRAEDTAVYFCSKVAAANNYYYALDVWGQGTTVTVSS

SEQ ID NO: 82 - protein, 112 aa, Artificial Sequence
  synthetic construct; antigen binding domain
DIVMTQSPLSLPVTPGEPASISCRSSQSLLHSNGYKYLDWYLQKPGQSPQLLIYLVSNRASGVPDRFSGSGSGTDFTLKISRVEAEDVGVYYCMQALQTPYTFGQGTKLEIK

SEQ ID NO: 83 - protein, 127 aa, Artificial Sequence
  synthetic construct; antigen binding domain
QVQLVESGGGVVQPGRSLRLSCVASGFTFSNYGMHWVRQAPGKGLEWVAVIWNDGSNKYYADSVKGRFTISRDNSKNTLYLQVSSLRADDTAVYYCARDGEVEYSSSNYNYYGLDVWGQGTTVTVSS

SEQ ID NO: 84 - protein, 107 aa, Artificial Sequence
  synthetic construct; antigen binding domain
DIQMTQSPSSLSASVGDRVTITCQASQDISNYLNWYQQKPGKAPKLLIYDASNLETGVPSRFSGSGSGTDFTFTISSLQPEDIVTYYCQQYDDLPITFGQGTRLEIK

SEQ ID NO: 85 - protein, 125 aa, Artificial Sequence
  synthetic construct; antigen binding domain
EVQLVESGGGLVQPGGSLRLSCAASGFSFHNFAMNWVRQAPGKGLEWVSVITGSGTSTHYADSVKGRFTISRDNSKKTLYLQMNSLRAEDTAVYYCAKDRGYDYSGSYYNWFDPWGQGTLVTVSS

SEQ ID NO: 86 - protein, 109 aa, Artificial Sequence
  synthetic construct; antigen binding domain
DIQMTQSPSSLSASVGDRITITCRASQSISSYLNWYQQKPGKAPKLLIFAASNLQSGVPSRFSGSGSGTDFTLTISSLQPEDFATYYCQQSYSTPSLFTFGPGTKVDIK

SEQ ID NO: 87 - protein, 128 aa, Artificial Sequence
  synthetic construct; antigen binding domain
EVQLVESGGGLVQPGGSLRLSCAVSGFTFSSYEMNWVRQAPGKGLEWVSHISSSGSTIYYADSVKGRFTMSRDNAKNSLYLQMNSLRAEDTAVYYCARDGNIWSGYYAAYYFYGMDVWGQGTTVTVSS

SEQ ID NO: 88 - protein, 112 aa, Artificial Sequence
  synthetic construct; antigen binding domain
DIVMTQTPLSSPVTLGQPASISCRSSQSLVHSDGKTYLSWLQQRPGQPPRLLIYKISNRFSGVPDRISGSGAGTDFTLKISRVEAEDVGVYYCMQAVQFPRTFGQGTKVEIK

SEQ ID NO: 89 - protein, 122 aa, Artificial Sequence
  synthetic construct; antigen binding domain
QVQLQQWGAGLLNPSETLSLTCAVYGGAFSDYYWNWIRQPPGKGLEWIGEINHRGSTNYNPSLKSRVTISVDTSKNQFSLRMSSVTAADAAVYYCARGEDYDIWNGYYQEKWGQGTLVTVSS

SEQ ID NO: 90 - protein, 107 aa, Artificial Sequence
  synthetic construct; antigen binding domain
EIVLTQSPATLSLSPGERATLSCRASQSISTYLAWYQQKPGQAPRLLIYDASKRATGIPARFSGSGSGTDFTLTISSLEPEDFVVYYCHQRSNWPLTFGGGTKVEIK

SEQ ID NO: 91 - protein, 117 aa, Artificial Sequence
  synthetic construct; antigen binding domain
QVQLQESGPGLVKPSETLSLTCTVSGGSFSSYYWSWLRQPPGKGLEWIGYIFYSGSTDYNPSLKSRVTISVDTSKKQFSLKLTSVTAADTAVYYCARTISTWWFAPWGQGTLVTVSS

SEQ ID NO: 92 - protein, 106 aa, Artificial Sequence
  synthetic construct; antigen binding domain
EIVMTQSPATLSVSPGGRATLSCRASQSVSNNVAWYQQKPGQAPRLLIYGASTRATGIPGRFSGSGSGTEFTLTISSLQSEDFAVYSCQQYNNWLTFGGGTKVEIK

SEQ ID NO: 93 - protein, 123 aa, Artificial Sequence
  synthetic construct; antigen binding domain
QVQLVESGGGVVQPGRSLRLSCVASGFTFSSYGMHWVRQAPGKGLEWVAIIWYDGSNKYYADSVKGRFTISRDNSKNTQYLQMNSLRAEDTAVYYCASVATSGDFDYYGMDVWGQGTTVTVSS

SEQ ID NO: 94 - protein, 107 aa, Artificial Sequence
  synthetic construct; antigen binding domain
EIVLTQSPATLSLSPGERTTLSCRASQRISTYLAWYQQKPGQAPRLLIYDASKRATGIPARFSGSGSGTGFTLTISSLEPEDFAVYYCQQRSNWPLTFGGGTKVEIK

SEQ ID NO: 95 - protein, 119 aa, Artificial Sequence
  synthetic construct; antigen binding domain
EVQLVQSGAEVRKPGESLKISCKGSGYSFTNYWIVWVRQMPGKGLEWMGIIYPGDSDTRYSPSFQGQVTISADKSISTAYLQWSSLKASDTAMYYCARRDTIFPSYPLWGQGTLVTVSS

SEQ ID NO: 96 - protein, 112 aa, Artificial Sequence
  synthetic construct; antigen binding domain
DIVMTQSPLSLPVTPGEPASISCRSSQSLLNSNGYNFLDWYLQKPGQSPQLLIYLVSNRASGVPDRFSGSGSGTDFTLKISRVEAEDIGVYYCMQALQTPITFGQGTRLEIK

SEQ ID NO: 97 - protein, 120 aa, Artificial Sequence
  synthetic construct; antigen binding domain
QITLKESGPTLVKPTQTLTLTCTFSGFSLSTNGVGVGWIRQPPGKALEWLTLIYWNENKHYSPSLKNRITITKDTSKNQVVLTMTNLDPVDTATYYCVHRGWLGAIFAYWGQGTLVTVSS

SEQ ID NO: 98 - protein, 108 aa, Artificial Sequence; identical to SEQ ID NO: 12
  synthetic construct; antigen binding domain

SEQ ID NO: 99 - protein, 126 aa, Artificial Sequence
  synthetic construct; antigen binding domain
EVQLVESGGGLVQPGGSLRLSCAASGFTFTSYAMTWVRQAPGKGLEWVSDISGSGGRTYYADSVKGRFTISRDNSKNMLYLQMNILRAEDTAVYHCAKGTGQQVDLYNYYYALDVWGQGTTVTVSS

SEQ ID NO: 100 - protein, 129 aa, Artificial Sequence
  synthetic construct; antigen binding domain
QVQLVESGGGVVQPGRSLRLSCAASGFTFSYYGMHWVRQAPGKGLEWVAVIWYDGSNKHYADSVKGRFTISRDNSKNTLYLQMNSLRADDTAVYYCARDKGISGIKGGSYYYYYAMDVWGQGTTVTVSS

SEQ ID NO: 101 - protein, 120 aa, Artificial Sequence
  synthetic construct; antigen binding domain
EVQLVESGGGLVKPGGSLRLSCAASGFTFSNAWMTWVRQAPGKGLEWVGRIKNKIDGGTTDYAAPVKGRFTISRDDSKNTVYLQMNSLKTEDTAVYYCSTVDYNWYFDFWGRGTLVTVSS

SEQ ID NO: 102 - protein, 129 aa, Artificial Sequence
  synthetic construct; antigen binding domain
QVQLVESGGGVVQPGRSLRLSCAASGFTFSFFGMHWVRQAPGKGLEWVALIWYDGTNENYADSVKGRFTISRDNSKSTLYLQMNSLRAEDTAVYYCARDRGVATFTRGNYYYNYGMDVWGQGTTVTVSS

SEQ ID NO: 103 - protein, 129 aa, Artificial Sequence
  synthetic construct; antigen binding domain
QVQLVESGGGVVQPGRSLRLSCAASGFTFSFYGMHWVRQAPGKGLEGVAVIWYDGSNKYYADSVKGRFTISRDNSKNMLYLQMTSLRAEDTAVYYCARDSGKTGTGITGYSYYYGMDVWGQGTTVTVSS

SEQ ID NO: 104 - protein, 118 aa, Artificial Sequence
  synthetic construct; antigen binding domain
QLQLQESGPGLVKPSETLSLTCTVSGGSIITNSYYWGWIRQPPGKGLEWIGSIYYSGRTYYNPSLESRVTISVDTSKNQFSLKLTSVTAADTAIYYCAREGDPSLDPWGQGTLVTVSS

SEQ ID NO: 105 - protein, 108 aa, Artificial Sequence; identical to SEQ ID NO: 24
  synthetic construct; antigen binding domain

SEQ ID NO: 106 - protein, 121 aa, Artificial Sequence
  synthetic construct; antigen binding domain
EVQLVESGGDLVQPGGSLRLSCAASGFTFSTYAMNWVRQAPGKGLEWVSHISGSGGNSYSADSVKGRFTISRDNSKNTLYLQMNSLRAEDTAIYYCSLDIMATVGGLFAYWGQGTLVTVSS

SEQ ID NO: 107 - protein, 131 aa, Artificial Sequence
  synthetic construct; antigen binding domain
QVQLVESGGGVVQPGRSLRLSCVASGFIFSFYGMHWVRQAPDKGLEWVAVIWYDGSNEYYADSVKGRFTISRDNSKNTLYLQMNSLRAEDTAVYYCGRDQGISYYDILTGNYNYYYGVDVWGQGTTVTVSS

SEQ ID NO: 108 - protein, 119 aa, Artificial Sequence
  synthetic construct; antigen binding domain
QVQLQQWGAGLLKPSETLSLTCAVYGGSFSGYYWNWIRQPPGKGLEWVGEISHRGSTNYNPSLKSRVTISLDTSKNQFSLKLTSVTAADTAVYYCSRDEELEFRFFDYWGQGTLVTVSS

SEQ ID NO: 109 - protein, 107 aa, Artificial Sequence; identical to SEQ ID NO: 46
  synthetic construct; antigen binding domain

SEQ ID NO: 110 - protein, 124 aa, Artificial Sequence
  synthetic construct; antigen binding domain
EVQLVESGGGLVQPGGSLRLSCVASGFTFSLYAMTWVRQVPGKGLEWVSTISGSGGGTYYTDSVKGRFTISRDNSKNTLYLQMNSLRADDTAVFYCTKESTTGTYSYFYGMDVWGQGTTVTVSS

SEQ ID NO: 111 - protein, 107 aa, Artificial Sequence
  synthetic construct; antigen binding domain
DIQMTQSPSSLSASVGDRVTITCRASQTISSYLNWYQQKPGKAPKLLIYAASSLQSGVPSRFSGSGSGTDFTLTLSGLQPEDFATYYCQQSYSTPLTFGGGTKVEIK

SEQ ID NO: 112 - protein, 121 aa, Artificial Sequence
  synthetic construct; antigen binding domain
EVQLVESGGGLVQPGGSLRLSCAASGFTFSRFWMSWVRQAPGKGLEWVANINQDGTEKYYVDSVKGRFTISRDNAKNSLYLQMNSLRAGDTAVYYCANTYYDFWSGHFDYWGQGTLVTVSS

SEQ ID NO: 113 - protein, 107 aa, Artificial Sequence
  synthetic construct; antigen binding domain
DIQMTQSPSTLSASVGDRVTITCRASQSISNWLAWYQQKPGKAPKLLIYKASSLESGVPSRFSGSGSGTEFTLTISSLQPDDFATYYCQQYHSYSYTFGQGTKLEIK

SEQ ID NO: 114 - protein, 121 aa, Artificial Sequence
  synthetic construct; antigen binding domain
QEHLVESGGGVVQPGRSLRLSCEASGFTFSNFGMHWVRQAPGKGLEWVAALWSDGSNKYYADSVKGRVTISRDNSKNTLYLQMNSLRAEDTAVYYCARGRGAPGIPIFGYWGQGTLVTVSS

SEQ ID NO: 115 - protein, 107 aa, Artificial Sequence
  synthetic construct; antigen binding domain
DIQMTQSPSSLSASVGDRVTITCRASQGIRNDLGWYQQKPGKAPKRLIYTASSLQSGVPSRFSGSGSGTEFTLTISSLQPEDFATYYCLQHNSYPLTFGGGTKVAIK

SEQ ID NO: 116 - protein, 130 aa, Artificial Sequence
  synthetic construct; antigen binding domain
EVQLVESGGGLVKPGGSLRLSCAASGFTFSNAWMSWVRQAPGKGLEWVGRIKRKTDGGTTDYAAPVKGRFTISRDDSKNTLHLQMNSLKTEDTAVYYCTTDDIVVVPAVMREYYFGMDVWGQGTTVTVSS

SEQ ID NO: 117 - protein, 107 aa, Artificial Sequence
  synthetic construct; antigen binding domain
DIQMTQSPSSLSASVGDRVTITCRTSQGIRNDLGWYQQKPGKAPKRLIYAASSLQSGVPSRFSGSGSGTEFTLTISSLQPEDFATYYCLQHNNYPYTFGQGTKLEIK

SEQ ID NO: 118 - protein, 121 aa, Artificial Sequence
  synthetic construct; antigen binding domain
QVQLVQSGAEVKKPGASVQVSCKASGYSFTGYYIHWVRQAPGQGLEWMGWINPNSGTKKYAHKFQGRVTMTRDTSIDTAYMILSSLISDDTAVYYCARDEDWNFGSWFDSWGQGTLVTVSS

SEQ ID NO: 119 - protein, 112 aa, Artificial Sequence
  synthetic construct; antigen binding domain
DIVMTQTPLSSPVTLGQPASISCRSSQTLVHGDGNTYLSWIQQRPGQPPRLLIYKVSNQFSGVPDRFSGSGAGTDFTLKISRVEAEDVGLYFCMQATHFPITFGQGTRLEIK

SEQ ID NO: 120 - protein, 121 aa, Artificial Sequence
  synthetic construct; antigen binding domain
QVHLVQSGAEVKKPGASVKVSCKASGYTFTGYYIHWVRQAPGHGLEWMGWLNPNTGTTKYIQNFQGRVTMTRDTSSSTAYMELTRLRSDDTAVYYCARDEDWNYGSWFDTWGQGTLVTVSS

SEQ ID NO: 121 - protein, 112 aa, Artificial Sequence
  synthetic construct; antigen binding domain
DIVMTQTPLSSPVTLGQPASISCRSSPSLVHSDGNTYLSWLQQRPGQPPRLLIYKISNRFSGVPDRFSGSGAGTDFTLKISRVEAEDVGVYYCMQATHFPITFGQGTRLEIR

SEQ ID NO: 122 - protein, 120 aa, Artificial Sequence
  synthetic construct; antigen binding domain
EVQLVESGGGVVRPGGSLRLSCAASGFTFDDYGMTWVRQAPGRGLEWVSGIHWHGKRTGYADSVKGRFTISRDNAKKSLYLQMNSLKGEDTALYHCVRGGMSTGDWFDPWGQGTLVIVSS

SEQ ID NO: 123 - protein, 108 aa, Artificial Sequence
  synthetic construct; antigen binding domain
DIQMTQSPSSLSASLGDRVTITCRASQSINSYLNWYQQKPGKAPKLLIYVASSLQSGVPSRFSGSGSGTEFTLTISNLQPEDFATYYCQQSYSTPPITFGQGTRLEIK

SEQ ID NO: 124 - protein, 120 aa, Artificial Sequence
  synthetic construct; antigen binding domain
EVQLVESGGGVVRPGGSLRLSCAASGFTFDDYGMTWVRQVPGKGLEWVSGIHWSGRSTGYADSVKGRFTISRDNAKNSLYLQMNSLRAEDTALYYCARGGMSTGDWFDPWGQGTLVTVSS

SEQ ID NO: 125 - protein, 108 aa, Artificial Sequence
  synthetic construct; antigen binding domain
DIQMTQSPSSLSASVGDRVTITCRASQSISSYLNWYQQKPGKAPKLLIYVASSLQSGVPSRFSGSGSGTDFTLTISSLQPEDFATYYCQQSYSTPPITFGQGTRLEIK

SEQ ID NO: 126 - protein, 115 aa, Artificial Sequence
  synthetic construct; antigen binding domain
EVQLVESGGGLVQPGGSLRLSCAASGFTVGSNYMNWVRQAPGKGLEWVSVIYSGGSTYYADSVKGRFTISRLTSKNTLYLQMSSLRPEDTAVYYCARGIRGLDVWGQGTTVTVSS

SEQ ID NO: 127 - protein, 108 aa, Artificial Sequence
  synthetic construct; antigen binding domain
DIQMTQSPSSLSASVGDRVTITCRASQTINIYLNWYQQKPGRAPRLLIYAASSLQSGVPSRFSGSGSGTDFTLTISSLQPEDFATYYCHQSYSTPPITFGQGTRLEIK

SEQ ID NO: 128 - protein, 115 aa, Artificial Sequence
  synthetic construct; antigen binding domain
EERLVESGGDLVQPGGSLRLSCAASGITVGTNYMNWVRQAPGKGLEWVSVISSGGNTHYADSVKGRFIMSRQTSKNTLYLQMNSLETEDTAVYYCARGIRGLDVWGQGTMVTVSS

SEQ ID NO: 129 - protein, 108 aa, Artificial Sequence
  synthetic construct; antigen binding domain
DIQMTQSPSSLSASVGDRVTITCRASQSMSSYLNWYQQKPGRAPKLLIFAASSLQSGVPSRFSGSGSGTDFTLTISSLQPEDFATYYCQQSYSTPPITFGQGTRLEIK

SEQ ID NO: 130 - protein, 118 aa, Artificial Sequence
  synthetic construct; antigen binding domain
QVQLVQSGAEVKMPGSSVRVSCKASGGIFSSSTISWVRQAPGQGLEWMGEIIPVFGTVNYAQKFQDRVIFTADESTTTAYMELSSLKSGDTAVYFCARNWGLGSFYIWGQGTMVTVSS

SEQ ID NO: 131 - protein, 108 aa, Artificial Sequence
  synthetic construct; antigen binding domain
EIVLTQSPGTLSLSPGERATLSCRASQSFNFNYLAWYQQKPGQAPRLLIYGASSRATGIPDRFSGSGSGTDFTLTINRLEPEDFGVFYCQQYESAPWTFGQGTKVEIK

SEQ ID NO: 132 - protein, 115 aa, Artificial Sequence
  synthetic construct; antigen binding domain
EVQLVESGGDLVHPGRSLRLSCAASGFPFDEYAMHWVRQVPGKGLEWVSGISWSNNNIGYADSVKGRFTISRDNAKNSLYLQMNSLRPEDTAFYYCAKSGIFDSWGQGTLVTVSS

SEQ ID NO: 133 - protein, 105 aa, Artificial Sequence
  synthetic construct; antigen binding domain
DIQMTQSPSSLSASVGDRVTITCRASQSISSYLNWYQQKPGKLLIYAASSLQSGVPSRFSGGGSGTDFTLTISSLRPEDFATYYCQQSYCTPPITFGQGTRLEIK

SEQ ID NO: 134 - protein, 118 aa, Artificial Sequence
  synthetic construct; antigen binding domain
EVQLVESGGGVVQPGRSLRLSCAASGFTFSSYGMHWVRQAPGKGLEWVTLISYEGRNKYYADSVKGRFTISRDNSKNTLYLQMNSLRAEDTAVYYCAKDRTLYGMDVWGQGTTVTVSS

SEQ ID NO: 135 - protein, 121 aa, Artificial Sequence
  synthetic construct; antigen binding domain
QVTLRESGPALVKTTQTLTLTCTFSGFSLSTNRMCVTWIRQPPGKALEWLARIDWDGVKYYNTSLKTRLTISKDTSKNQVVLTMTNMDPVDTATFYCARSTSLTFYYFDYWGQGTLVTVSS

SEQ ID NO: 136 - protein, 108 aa, Artificial Sequence; identical to SEQ ID NO: 12
  synthetic construct; antigen binding domain

SEQ ID NO: 137 - protein, 115 aa, Artificial Sequence
  synthetic construct; antigen binding domain
EVQLVESGGGLVQPGGSLRLSCAASEFTVGTNHMNWVRQAPGKGLEWVSVIYSGGNTFYADSVKGRFTISRHTSKNTLYLQMNSLTAEDTAVYYCARGLGGMDVWGQGTTVTVSS

SEQ ID NO: 138 - protein, 107 aa, Artificial Sequence
  synthetic construct; antigen binding domain
DIQMTQSPSSLSASVGDRVTITCRASQVISNYLAWYQQKPGKVPRLLIYAASTLQSGVPSRFSGSGSGTDFTLTISSLQPEDVATYYCQKYNSAPRTFGQGTKVEIK

SEQ ID NO: 139 - protein, 120 aa, Artificial Sequence
  synthetic construct; antigen binding domain
EVQLVESGGGLVQRGESLRLYCAASGFTFSKYWMNWVRQAPGKGLEWVANIKGDGSEKYYVDSVKGRFTISRDNAKNSLYLQMNSLRAEDTAVYYCARDYWGSGYYFDFWGQGTLVTVSS

SEQ ID NO: 140 - protein, 107 aa, Artificial Sequence
  synthetic construct; antigen binding domain
DIQMTQSPSSLSASVGDRVTITCRASQNINNYLNWYQQKPGKAPKLLIYAASSFQNAVPSRFSGSGSGTDFTLTISSLQPEDFATYYCQQSYNTPLTFGGGTKVEIK

SEQ ID NO: 141 - protein, 130 aa, Artificial Sequence
  synthetic construct; antigen binding domain
EVQLVESGGGLVQSGGSLRLSCAASGFTFSSYWMSWVRQAPGKGLEWVANIKQDGSEKYYVDSVKGRFTISRDNAKNSLYLQMNSLRADDTAVYYCARDDIVVVPAPMGYYYYYFGMDVWGQGTTVTVSS

SEQ ID NO: 142 - protein, 107 aa, Artificial Sequence
  synthetic construct; antigen binding domain
DIQMTQSPSSLSASVGDRVTITCRASQGIRNDLGWYQQKPGKAPKRLIYAASSLQSGVPSRFSGSGSGTEFTLTISSLQPEDFATYYCLQHNSYPYTFGQGTKLEIK

SEQ ID NO: 143 - protein, 123 aa, Artificial Sequence
  synthetic construct; antigen binding domain
EVQLVESGGGLVQPGRSLRLSCAASGFTFDDFAMHWVRQAPGKGLEWVSGISWTGGNMDYANSVKGRFTISREDAKNSLYLQMNSLRAADTALYYCVKDIRGIVATGGAFDIWGRGTMVTVSS

SEQ ID NO: 144 - protein, 107 aa, Artificial Sequence
  synthetic construct; antigen binding domain
DIQMTQSPSSLSASVGDRVTISCRASQTISTYLNWFQQKPGKAPKLLIYVVSSLQSGVPSRFSGSGSGTDFTLTISSLQPEDFATYYCQQSYSTPFTFGPGTKVDIK

SEQ ID NO: 145 - protein, 115 aa, Artificial Sequence
  synthetic construct; antigen binding domain
EVQLVESGGGLVQPGGSLRLSCAASGFTVGTNYMNWVRQAPGKGLEWISVIYSGGSTFYADSVKGRFTISRQTSQNTLYLQMNSLRPEDTAVYYCARGIRGFDIWGQGTMVTVSS

SEQ ID NO: 146 - protein, 108 aa, Artificial Sequence; identical to SEQ ID NO: 12
  synthetic construct; antigen binding domain

SEQ ID NO: 147 - protein, 115 aa, Artificial Sequence
  synthetic construct; antigen binding domain
EVQLVESGGGLVQPGGSLRLSCAASGFTISTNYMNWVRQAPGKGLEWVAVIYSSGSTYYIDSVKGRFTISRLTSKNTVYLQMSSLNSEDTAVYYCARGIRGFDIWGQGTMVTVSS

SEQ ID NO: 148 - protein, 124 aa, Artificial Sequence
  synthetic construct; antigen binding domain
EVQLVESGGGLVQPGRSLRLSCAASGFTIDDSAMHWVRQTPGKGLEWVSGISWKSGSIGYADSVRGRFTISRDNAKNSLYLQMNSLRVEDTALYYCVKDIRGNWNYGGNWFDPWGQGTLVTVSS

SEQ ID NO: 149 - protein, 115 aa, Artificial Sequence
  synthetic construct; antigen binding domain
EVQLVESGGGLVQPGGSLRLSCEASGFTVGVNHMNWVRQAPGKGLEWVSVIFSSGRTFYGDYVKGRLTIFRQTSQNTVYLQMNSLRSEDTAIYYCARGIGGLDIWGRGTMVTVSS

SEQ ID NO: 150 - protein, 123 aa, Artificial Sequence
  synthetic construct; antigen binding domain
EVQLVESGGGLVQPGRSLRLSCAASGFTFDDYALHWVRQAPGKGLEWVSGISWTGGTIDYADSVKGRFTISRDNAKNSLYLQMSSLRTEDTAIYYCTRDIRGNWKYGGWFDPWGQGTLVTVSS

SEQ ID NO: 151 - protein, 120 aa, Artificial Sequence
  synthetic construct; antigen binding domain
QVQLVQSGTEVKKPGASVKVSCKASGYTFTAYYMHWVRQAPGQGLDWMGWISPNSGFTNYAQKFQGRVTMTRDTSINTFYMELSGLRSDDTAVYYCAREGSTHHNSFDPWGQGTLVTVSS

SEQ ID NO: 152 - protein, 114 aa, Artificial Sequence
  synthetic construct; antigen binding domain
EVQLVESGGGLVQPGGSLRLSCAASGFTVGTNFMNWVRQAPGKGLEWVSAIYSGGTANYADSVKGRFTISRDTSRNTLYLQMNSLRTEDTAVYYCARGGGMDVWGQGTTVTVSS

SEQ ID NO: 153 - protein, 118 aa, Artificial Sequence
  synthetic construct; antigen binding domain
QVQLVQSGAEVKKPGSSVKVSCKASGGTFNTYVLSWVRQAPGQGLEWMGEIIPILGAANYAQNFQGRVTFTTDESTNTAYMDLSSLRSEDTAVYYCARDRTSGGFDPWGQGTLVTVSS

SEQ ID NO: 154 - protein, 119 aa, Artificial Sequence
  synthetic construct; antigen binding domain
QVQLVQSGAEVEKPGASVKVSCKASGYIFTHYGISWVRQAPGQGLEWVGWISPYNGYTDYAQKLQGRVTLTTDTSTTTAYMELRNLRSDDTAMYYCSRGRGPYWSFDLWGRGTLVTVSS

SEQ ID NO: 155 - protein, 117 aa, Artificial Sequence
  synthetic construct; antigen binding domain
QVQLVQSGAEVKKPGASVKVSCKASDYTFTSYGISWVRQAPGQGLEWMGWISVYNGNINYAQKFKGRVTMTTDTSTSTAYMELRSLRSDDMAVYYCARVTQFGMDVWGQGTTVTVSS

SEQ ID NO: 156 - protein, 107 aa, Artificial Sequence
  synthetic construct; antigen binding domain
DIQMTQSPSSLSASVGDRVTITCRASQSISSNLNWYQQNPGKAPKLLIYTTSSLQGGVPSRFSGSGSGTDFTLTISSLQPEDFATYYCQQSFRTPFTFGPGTKVDIK

SEQ ID NO: 157 - protein, 128 aa, Artificial Sequence
  synthetic construct; antigen binding domain
EVQLVESGGGLVQPGGSLKLSCAASGFTFSGSAMHWVRQASGKGLEWVGRIRGKANSFATAYSASVKGRFTISRDDSKNTASLQMNSLRTEDTAVYFCTREDQQLVRPYYYHYGMDVWGQGTTVTVSS

SEQ ID NO: 158 - protein, 107 aa, Artificial Sequence
  synthetic construct; antigen binding domain
DIQMTQSPSSLSASVGDRVTITCRTSQSITNYLNWYQQKPGKAPKLLIYATASLQSGVPSRFSGSGSETDFTLTISSLQPEDFATYYCQQSYSTPLTFGGGTKVEIK

SEQ ID NO: 159 - protein, 123 aa, Artificial Sequence
  synthetic construct; antigen binding domain
QITLKESGPTLVKPTQTLTLTCTFSGFSLSTSGVGVGWIRQSPGRALEWLALIYWNDHERYSPSLKSRLTITKDTSKNLVVLAMANMDPVDTATYFCAHRNIEYRRSYFFDYWGQGTLVTVSS

SEQ ID NO: 160 - protein, 107 aa, Artificial Sequence
  synthetic construct; antigen binding domain
DIQMTQSPSSVSASVRDRVTVTCRASQDINNWLAWYQQKPGKAPKLLIYAASSLQSGVPSRFSGSGSGTDFTLTISSLQPEDFATYYCQQANTFPFTFGPGTKVDIK

SEQ ID NO: 161 - protein, 118 aa, Artificial Sequence
  synthetic construct; antigen binding domain
QVQLQESGPGLVKPSETLSLTCTVSGGSINSYYWTWIRQPPGKGLEWIGYVYYSGSTTYNPSLKSRVTISVDTSKNQFFLNLNSVTAAETAVYYCARGTLGYYGMDVWGQGTTVTVSS

SEQ ID NO: 162 - protein, 108 aa, Artificial Sequence
  synthetic construct; antigen binding domain
EIVLTQSPGTLSLSPGERATLSCRASQSFSNNYLAWYQQKPGQAPRLLIYGTSIRATGIPDRFSGSGSGTDFTLAISRLEPEDFAVYYCQQYGRSPLTFGGGTKVEIK

SEQ ID NO: 163 - protein, 118 aa, Artificial Sequence
  synthetic construct; antigen binding domain
QVQLVESGGGVVQPGRSLRLSCAASGFTFSSYGMNWVRQAPGKGLEWVAVTWYDGSNKHYADSVKGRFTISRDNSKNTLYLQMYSLRAEDTAMYYCVRGGHLGAFDIWGQGTMVTVSS

SEQ ID NO: 164 - protein, 107 aa, Artificial Sequence
  synthetic construct; antigen binding domain
EIVLTQSPGTLSLSPGERATLSCRASQSVSSYLAWYQQKPGQAPRLLIYGASSRATGIPDRFSGGGSGTDFTLTISRLEPEDFAVYYCQQYGSSPFTFGPGTKVDIK

SEQ ID NO: 165 - protein, 121 aa, Artificial Sequence
  synthetic construct; antigen binding domain
QVQLVQSGAEVKKPGASVKVSCKASGYTFTDYYIHWVRQAPGQGLEWMGWINPNNGVSNYAQKFQGRVTMTRDTSISTAYMDLIRLRSDDTAVYYCARERASWDYNGVDVWGQGTTVTVSS

SEQ ID NO: 166 - protein, 112 aa, Artificial Sequence
  synthetic construct; antigen binding domain
DIVMTQSPLSLPVTPGEPASISCRSSQSLLHSNGYSYLDWYLQKPGQSPQLLIYLGSNRASGVPDRFSGSGSGTDFTLKISRVEAEDVGVYYCMQGLQPPNTFGQGTKLEIK

SEQ ID NO: 167 - protein, 118 aa, Artificial Sequence
  synthetic construct; antigen binding domain
QLQLQESGPGLVKPSETLSLTCIVSGGSTSSNTYYWGWIRQPPGKGLEWIGTIHYSGNPYYDPSLKSRVTISVDTSKNHFSLKLNSVTAADTAVYYCTRQYINFFDFWGQGTLVTVSS

SEQ ID NO: 168 - protein, 107 aa, Artificial Sequence
  synthetic construct; antigen binding domain
EIVLTQSPATLSLSPGERVTLSCRASQSISRYLAWYQQKPGQAPRVLIYDASNRATDIPARFSGSGSGTDFTLTISSLEPEDFAVYYCQQRSNWPITFGQGTRLEIK

SEQ ID NO: 169 - protein, 121 aa, Artificial Sequence
  synthetic construct; antigen binding domain
QVQLVESGGGVVQPGRSLRLSCAASGLTFSYYGMHWVRQAPGKGLEWVAVISYDGSNKYYADSVKGRFTISRDNSKNTLYLQMNSLRAEDAAVYYCAKDLGGDDYYGMDVWGQGTTVTVSS

SEQ ID NO: 170 - protein, 108 aa, Artificial Sequence
  synthetic construct; antigen binding domain
EIVLTQSPGTLSLSPGERATLSCRASQSVSRTYLAWYQQKPGQAPRLLIYGAFSRATGIPDRFSGSGSGTDFTLTISRLEPEDFAVYYCQQYGSSPYTFGQGTKLEIK

SEQ ID NO: 171 - protein, 122 aa, Artificial Sequence
  synthetic construct; antigen binding domain
QVQLVESGGGLVKPGGSLRLSCAASGFTFSDYYMTWIRQAPGKGLEWVSYISSSGGNIFYADSVKGRFTISRDNAKNSLYLQMNSLRGEDTAVYYCARGLEPYHYYYGMDVWGQGTTVTVSS

SEQ ID NO: 172 - protein, 107 aa, Artificial Sequence
  synthetic construct; antigen binding domain
DIQMTQSPSSLSASVGDRVTITCQASQDISNYLNWYQQKPGKAPKLLIYDASNLETGVPSRFSGSGSGTDFTFTISSLQPEDIATYFCQHYDNLPFTFGPGTKVDIK

SEQ ID NO: 173 - protein, 123 aa, Artificial Sequence
  synthetic construct; antigen binding domain
EVQLVESGGGLVQPGGSLRLSCAASGFTLSNYVMTWVRQAPGKGLEWVSAISGRGGNSYYADSVKGRFSISRDHSKNTLYLQVNSLRAEDTAVYYCAKAERGYSYGFNWFDPWGQGTLVTVSS

SEQ ID NO: 174 - protein, 107 aa, Artificial Sequence
  synthetic construct; antigen binding domain
DIQMTQSPSSVSASAGDRVTITCRASQGISSWLAWYQQKPGKAPKLLIYAASSLQSGVPSRFSGSGSGTDFTLTISSLQPEDFASYYCQQGNNFPLTFGGGTKVEIK

SEQ ID NO: 175 - protein, 120 aa, Artificial Sequence
  synthetic construct; antigen binding domain
QVQLVESGGGVVQPGRSLRLSCAASGFTFSTYGMHWVRQAPGKGLEWVTVIWYDGNNKYYADSVKGRFTISRDNSKNTLYLQMNNLRAEDTALYYCARGGGRLSYYHDYWGQGTLVTVSS

SEQ ID NO: 176 - protein, 107 aa, Artificial Sequence
  synthetic construct; antigen binding domain
DIQMTQSPSSLSASVGDRVTITCRASQSISTFLNWYQQKPGKAPNLLIYGTSSLQSGVPSRFSGSGSGTDFTLTISSLQPEDFAAYYCQQTYSTPFTFGPGTKVDIK

SEQ ID NO: 177 - protein, 119 aa, Artificial Sequence
  synthetic construct; antigen binding domain
QVQLVQSGAEVKMSGASVRVSCKASGYTFTSYGISWMRQAPGQGLEWMGWITAYNGNSNYAQKLQGRVTMTTDTSTGTAYMELRSLTSDDTAVYYCARRGDYLGVFPYWGQGTLVTVSS

SEQ ID NO: 178 - protein, 107 aa, Artificial Sequence
  synthetic construct; antigen binding domain
DIQMTQSPSSLSASVGDRVTITCRASQSISSYLNWYQQKPGKAPNLLIYTASSLQSGVPSRFSGSGSGTDFTLTISSLQPEDFATYYCQQSYSSPLTFGGGTKVEIK

SEQ ID NO: 179 - protein, 116 aa, Artificial Sequence
  synthetic construct; antigen binding domain
EVQLVESGGGLVQPGGSLRLSCAASGFTFSNYEMSWVRQAPGKGLEWVSSIRTSGTTKYYADSMKGRFTISRDNAKNSLYLQMNSLRAEDTAVYYCAGGGTFLHYWGQGTLVTVSS

SEQ ID NO: 180 - protein, 108 aa, Artificial Sequence
  synthetic construct; antigen binding domain
DIQMTQSPSSVSASVGDRVTITCRASQGIASYLAWYQQKPGKAPKLLIYAASSLQTGVPSRFSGSGYGTDFTLTISSLQPEDFATYYCQQAKSFPMYTFGQGTKLEIK

SEQ ID NO: 181 - protein, 122 aa, Artificial Sequence
  synthetic construct; antigen binding domain
QVQLQESGPGLVKPSQTLSLTCTVSGGSITSGGYYWSWIRQHPGKGLEWIGYIFYSGITNYNPSLKSRVTISVDTSKNQFSLKLTSVTAADTAVYYCATYNSLRLYYGMDVWGQGTTVTVSS

SEQ ID NO: 182 - protein, 112 aa, Artificial Sequence
  synthetic construct; antigen binding domain
DVVMTQSPLSLPVILGQPASISCRSSQSLVYGDGNTYLNWFQQRPGQSPRRLIYKVSNRDSGVPDRFSGSGSGTDFTLKISRVEAEDVGVYYCMQSTHWPLTFGGGTKVEIK

SEQ ID NO: 183 - protein, 120 aa, Artificial Sequence
  synthetic construct; antigen binding domain
EVQLVESGGGLVQPGGSLRLACAASGFTFSDYYMDWVRQVPGKGLEWVGRSRDKANSFTTEYVASVKGRFTISREDSKNSVYLQMNSLKTEDTAVYYCARTNYDFSLDVWGQGTTVTVSS

SEQ ID NO: 184 - protein, 107 aa, Artificial Sequence
  synthetic construct; antigen binding domain
DIQMTQSPSSLSASVGDRVTITCRASQDINNYLAWFQQKPGNAPKSLIYAASSLQSGVPSKFSGSGSGTDFTLTISSLQPEDFATYYCQQYSTYPITFGQGTRLEIK

SEQ ID NO: 185 - protein, 118 aa, Artificial Sequence
  synthetic construct; antigen binding domain
QVQLQESGPGLVKPSETLSLTCTVSGGSISSYHWSWIRQPLGKGLEWIGYIYYSGSTNYNPSLKSRVTISVDTSKNQFSLKLSSVTAADTAVYYCARGGSSIWPFDYWGQGTLVTVSS

SEQ ID NO: 186 - protein, 107 aa, Artificial Sequence
  synthetic construct; antigen binding domain
DIQMTQSPSTLSASVGDRVTITCRASQSISSWLAWYQQKSGKAPKLLISKASTLESGVPSRFSGSGSGTEFTLTISSLQPDDFATYYCQQYNIYSWTFGQGTKVEIK

SEQ ID NO: 187 - protein, 120 aa, Artificial Sequence
  synthetic construct; antigen binding domain
QITLKESGPTLVKPTQTLTLTCTFSGFSLSTSGVGVGWIRQPPGVALEWLALIYWNDDKRFSPSLKSRLTITKDTSKNQVVLTMTNMDPVDTATYYCAHRRLGLYYFDYWGQGTLVTVSS

SEQ ID NO: 188 - protein, 107 aa, Artificial Sequence
  synthetic construct; antigen binding domain
DIQLTQSPSFLSASVGDRVTITCWASQGISSYLAWYQQKPGKAPKLLIYAASTLQSGVPSRFSGSGSGTEFTLTISSLQPEDFATYYCQQVHIYPFTFGPGTKVDIK

SEQ ID NO: 189 - protein, 122 aa, Artificial Sequence
  synthetic construct; antigen binding domain
QVQLVQSGAEVKKPGASVKVSCKASGYTLSSYGISWVRQAPGQGLEWMGWISAYNGNTNYAQKLQGRLTMTTDTSTSTAYMELRSLRSDDTAVYYCSRDGPFKISFFGMDVWGQGTTVTVSS

SEQ ID NO: 190 - protein, 108 aa, Artificial Sequence; identical to SEQ ID NO: 12
  synthetic construct; antigen binding domain

SEQ ID NO: 191 - protein, 118 aa, Artificial Sequence
  synthetic construct; antigen binding domain
QVQLVESGGGEVQPGRSLRLSCAASGFTFSSYGMHWVRQAPGKGLEWVAVIWYDGRNKHYVDSVKGRFTISRDNSKNTVYLQMNSLRAEDSAVYYCVRGGQLGAFDYWGQGTLVTVSS

SEQ ID NO: 192 - protein, 108 aa, Artificial Sequence; identical to SEQ ID NO: 24
  synthetic construct; antigen binding domain

SEQ ID NO: 193 - protein, 118 aa, Artificial Sequence
  synthetic construct; antigen binding domain
QVQLVESGGGVVQPGRSLRLSCAASGFTSSSYGIHWVRQAPGKGLEWVAVIWYDGSNKYYADSVKGRFTISRDNSKNTLYLQMNSLRAEDTAVYYCARGGPWGAFDIWGQGTMVTVSS

SEQ ID NO: 194 - protein, 108 aa, Artificial Sequence
  synthetic construct; antigen binding domain
DIRMTQSPSSLSASVGDRVTITCRASQTVNTFLNWYQQKPGKAPKLLIFGASSLQSGVPSRFSGSGSGTDFTLTISGLQPEDFAIYYCQQSYSVPPITFGQGTRLEIE

SEQ ID NO: 195 - protein, 122 aa, Artificial Sequence
  synthetic construct; antigen binding domain
QVQLHESGPGLVKPSQTLSLTCSVSGGSISNGGYYWSWIRQHPGQGLEWIGYIYYIGNTYYNPSLESRVTMSIDTSKNQFSLKLSSVTAADTAIYYCARQEFVPGAEYFLHWGQGILVTVSS

SEQ ID NO: 196 - protein, 107 aa, Artificial Sequence
  synthetic construct; antigen binding domain
DIQMTQSPSSLSASVGDRVTITCRASQDIRNDLGWHQQKSGKAPKSLIYAASSLQSGAPSRFSGSGSGTEFTLTISSLQPEDSATYYCLQQNSYPPTFGQGTKVEIK

SEQ ID NO: 197 - protein, 122 aa, Artificial Sequence
  synthetic construct; antigen binding domain
EVQLVESGGGLVQPGRSLRLSCAGTGFIFDDYAMHWVRQAPGKGLEWVSGISWNSNSLGYADSVKGRFTISRDNAKKSLYLQMSSLRAEDTALYYCVKDVTRLELRGFLDYWGQGTQVTVSS

SEQ ID NO: 198 - protein, 108 aa, Artificial Sequence
  synthetic construct; antigen binding domain
EIVLTQSPDTLSLSPGERATLSCRASQSVSSSFLAWYQQKPGQAPRLLIYGASSRATGIPDRFSGSGSGTDFTLTISRLEPEDFAVYYCQQYGRSPWTFGQGTKVAIK

SEQ ID NO: 199 - protein, 118 aa, Artificial Sequence
  synthetic construct; antigen binding domain
DRQMVESGGGVVQPGRSLRLSCIASGFIISRYGMHWVRQAPGKGLEWVAVIWYDGRNKNYADSVKGRFTISRDNSKNTLYLEMNSLRAEDTAVYYCGRVHQFGAFDIWGQGTMVTVSS

SEQ ID NO: 200 - protein, 108 aa, Artificial Sequence
  synthetic construct; antigen binding domain
DIQMTQSPSSLSASVGDRITITCRGSQNIGSFLSWYQQRPGKAPKLLIFGAYNLQGGVPSRFSGSGSGTDFTLTISSLQPEDFATYFCQQSYSTPPITFGQGTRLEIK

SEQ ID NO: 201 - protein, 121 aa, Artificial Sequence
  synthetic construct; antigen binding domain
QVQLQESGPGLVKPSQTLSLTCTVSGGSINNGGHYWTWIRQHPGKGLEWIGYIYYIGTTYYNPSLESRLSLSVDTSKNQFSLKLSSVTAADTAIYYCARSSLSVSEAFDVWGQGTMVTVSS

SEQ ID NO: 202 - protein, 108 aa, Artificial Sequence
  synthetic construct; antigen binding domain
DIQMTQSPSSLSASVGDRFTITCRASQSIGSFLSWYQQKPGKAPKLLIYAASSLQSGVPSRFSGSGSGTDFTLTISSLQPEDFATYYCQQSYNTPPITFGQGTRLEIK

SEQ ID NO: 203 - protein, 121 aa, Artificial Sequence
  synthetic construct; antigen binding domain
QVQLQESGPGLVRPSQTLSLTCTVSGGSISNGGYYWTWIRQNPGKGLEWIGYIYYIGTTYYNPSLESRLSLSVDTSKNQFSLKLTSVTAADTAVYYCARSSLAVSEAFDIWGQGTMVTVSS

SEQ ID NO: 204 - protein, 108 aa, Artificial Sequence
  synthetic construct; antigen binding domain
DIQLTQSPSSLSASVGDRVTITCRASQTISTYLNWYQQKPGNAPKLLIYAASSLQSGVPSRFSGRGSGTDFTLTISSLQPEDFATYYCQQGYTTPPITFGQGTRLEIK

SEQ ID NO: 205 - protein, 121 aa, Artificial Sequence
  synthetic construct; antigen binding domain
QVQLVQSGTEVKRPGASVKVSCKASGFTFTGYYIYWVRQAPGEGLEWMGWINPHSGGTKYAQKFQGRVTLTRDTSINTAYLDLISLRSDDTAVYYCARIGGGGYSSYFDYWGQGTLVTVSS

SEQ ID NO: 206 - protein, 107 aa, Artificial Sequence
  synthetic construct; antigen binding domain
DIQMTQSPSSVSASVGDRVTITCRASQDISSWLAWYQQKPGKAPKLLIYTTANLQSGVPSRFSGSGSGTDFTLTISSLQSEDFATYYCQQANSFPFTFGSGTKVDIK

SEQ ID NO: 207 - protein, 121 aa, Artificial Sequence
  synthetic construct; antigen binding domain
EVQLLESGGGLVQPGGSLRLSCAASGFTFSSYAMSWVRQAPGKGLEWVSDISGSGLSTYYADSVKGRFAISRDNSKNMLYLQMNRLRAEDTAVYYCAKEPSHWNGEAFDIWGQGTMVTVSS

SEQ ID NO: 208 - protein, 108 aa, Artificial Sequence
  synthetic construct; antigen binding domain
EIVLTQSPDTLSLSPGERATLSCRASQTVSNSHLAWYQQKPGQAPRLLIYGTSSRATGIPDRFSGSGSGTDFSLTIIRLEPDDFAVYFCQQHESSPPTFGQGAKLEIK

SEQ ID NO: 209 - protein, 122 aa, Artificial Sequence
  synthetic construct; antigen binding domain
QLQLQESGPGLVKPSETLSFTCTVSGGSISSNYYYWGWVRQSPGKGLEWIGSIYHTGNAYDNPSLKSRVTISVDTSKNQFSLNLNSVTAADTAIYYCARHHSSSSWWYFDVWGRGTLVIVSS

SEQ ID NO: 210 - protein, 108 aa, Artificial Sequence
  synthetic construct; antigen binding domain
EIVLTQSPGTLSLSPGERATLSCRASQWISSSYLAWYQQKPGQAPRLLIYGAFSRAPGIPGRFSGSGSGTDFTLTISRLEPEDFAVYYCQQYGSSPYTFGQGTKLEIN

SEQ ID NO: 211 - protein, 121 aa, Artificial Sequence
  synthetic construct; antigen binding domain
QVQLVESGGGVVQPGRSLRLSCAASGITFSSYGMHWVRQAPGKGLEWVALTSYDGSKKYYSDSVKGRFTISRDNSKNTLYLQMNSLRPEDTAVYYCAKDKGGDDYYGMDVWGQGTTVTVSS

SEQ ID NO: 212 - protein, 108 aa, Artificial Sequence
  synthetic construct; antigen binding domain
DIQMTQSPSSLSASVGDRVTITCRASQSISTYLNWYQQKPGKAPKLLIYAASTLQSGVPSRFGGSGSGTDFTLTVSSLQPEDFATYYCQQSYSTPPITFGQGTRLEIN

SEQ ID NO: 213 - protein, 122 aa, Artificial Sequence
  synthetic construct; antigen binding domain
QVQLVQSGAEVKKPGASVKVSCKTSGYTFTNNGISWVRQVPGQGLEWMGWISPYNGNTKYAQKFQGRVTMTTDTSTTTVYMDVRSLRSDDTAVYFCARDGPITISYFGMDVWGQGTTVTVSS

SEQ ID NO: 214 - protein, 108 aa, Artificial Sequence
  synthetic construct; antigen binding domain
EIVLTQSPDTLSLSPGERATLSCRASQSVAGSYLAWYQQKPGQAPRLLIYGASSRATGIPDRFSGSGSGTDFTLTISRLEPEDFAVYYCQQYGTSPWTFGQGTKVEIT

SEQ ID NO: 215 - protein, 118 aa, Artificial Sequence
  synthetic construct; antigen binding domain
QVQLVESGGGVVQPGRSLRLSCAASGFTVNRYGIHWVRQAPGKGLEWVAVTWYDGRNKYFADSVKGRFSFSRDSSTNTLYLQMNSLRAEDTAVYYCARGGLFGYFDYWGQGTLVTVSS

SEQ ID NO: 216 - protein, 107 aa, Artificial Sequence
  synthetic construct; antigen binding domain
EIVLTQSPGTLSLSPGERATLSCRASQSVSSYLAWYQQKPGQAPRLLIYGASSRATGIPDRFSGSGSGTDFILTINRLEPEDFAVYYCQHYGNSPWTFGQGTKVEIK

SEQ ID NO: 217 - protein, 118 aa, Artificial Sequence
  synthetic construct; antigen binding domain
QVQLVESGGGVVQPGRSLRLSCAASGFTFSSYGIHWVRQAPGKGLEWVAVIWYGGNNKYYADSVKGRFTISRDNSKNTLYLQMNSLRAEDTALYHCARSGNFGAFDIWGQGTMVTVSS

SEQ ID NO: 218 - protein, 123 aa, Artificial Sequence
  synthetic construct; antigen binding domain
QVQLVESGGGVVQPGRSLRLSCAASGFTFSSYGMDWVRQAPGKGLEWVAVIWYPGSNKYYADSVKGRFTVSRDNSKNTLYLQMNSLRAEDTAVYYCARDGELGLDYYSGMDVWGQGTTVTVSS

SEQ ID NO: 219 - protein, 107 aa, Artificial Sequence
  synthetic construct; antigen binding domain
DIQMTQSPSSLSASVGDRVTITCRASQGIRNDLNWYQQKPGKAPKRLINGASSLQSGVPSRFSGSGSGTEFTLTISSLQPEDFATYYCLQLNSYPRTFGQGTKVEIK

SEQ ID NO: 220 - protein, 123 aa, Artificial Sequence
  synthetic construct; antigen binding domain
QVQLVESGGGVVQPGRSLRLSCAASGFTFSNYGMHWVRQAPGKGLEWVAVIWYPGSNKFYTDSVEGRFTISRDNSKNTVYLQMDSLRAEDTAVYYCARGGALGVDYYYGMDVWGQGTTVTVSS

SEQ ID NO: 221 - protein, 107 aa, Artificial Sequence
  synthetic construct; antigen binding domain
AIQMTQSPSSLSASVGDRVTLTCRASQGIRNDLGWYQQKPGKAPNFLIYSASSLQSGVPSRFSGSGSGTDFTLTISSLQPEDFATYYCLQNYNYPWTFGQGTKVEIK

SEQ ID NO: 222 - protein, 124 aa, Artificial Sequence
  synthetic construct; antigen binding domain
QVQLVESGGGVVQPGRSLRLSCVASGFTFSDYGMHWVRQAPGKGLEWVAVIWYEGSNKYYADSVTGRFTISRDNSKNTLFLQMNSLKAEDTAEYYCAKDGGQLAYQYYYGMDVWGQGTTVTVSS

SEQ ID NO: 223 - protein, 107 aa, Artificial Sequence
  synthetic construct; antigen binding domain
AIQMTQSPSSLSASVGDRVTLTCRASQGIRNDLGWYQQKPGKAPKSLIYAASNLQSGVPSRFSGSGSGTDFTLTISSLQPEDSATYYCLQDYNYPRTFGQGTKVEIK

SEQ ID NO: 224 - protein, 123 aa, Artificial Sequence
  synthetic construct; antigen binding domain
QVQLVESGGGVVQPGRSLRLSCAASGFNFRSYGMHWVRQAPGKGLEWVAVIWYDGSNKYYADSVKGRFTISRDSSRDTLFLQMNSLRAGDTAVYYCARGGMLGRDYYYGMDVWGQGTTVTVSS

SEQ ID NO: 225 - protein, 107 aa, Artificial Sequence
  synthetic construct; antigen binding domain
DIQMTQSPSSLSASVGDRVTITCRASQGIRNDLGWYQQKPGKAPKRLIYAASSLQSGVPSRFSGSGSGTEFTLTISSLQPEDFATYYCLQHNSYPNTFGQGTKLEIK

SEQ ID NO: 226 - protein, 123 aa, Artificial Sequence
  synthetic construct; antigen binding domain
QVQLVESGGGAVQPGTSLRLSCAASGFTFSSFGMHWVRQAPGKGLEWVSVIWYEGSNKYYADSVKGRFTISRDNSRNTLSLQMDSLRVEDTAVYYCARGGELGVNYYYDMDVWGQGTTVTVSS

SEQ ID NO: 227 - protein, 107 aa, Artificial Sequence
  synthetic construct; antigen binding domain
DIQMTQSPSSLSASVGDRVTITCRASQDIKNDLGWFQQKAGKAPKRLFYATSSLQSGVPSRFSGSGSGTEFTLTISSLQPEDFATYYCLQVHSYPRTFGQGTKVEIK

SEQ ID NO: 228 - protein, 123 aa, Artificial Sequence
  synthetic construct; antigen binding domain
QVQLVESGGGVVQPGRSLRLSCEASGFTFSNYGFHWVRQAPGKGLDWVAVIWYAGSNKFYVDSVQGRFTISRDNSKQILFLQMNSLRAEDSAVYYCVRGGILGIDYYSGMDVWGQGTTVTVSS

SEQ ID NO: 229 - protein, 107 aa, Artificial Sequence
  synthetic construct; antigen binding domain
AIQMTQSPSSLSASVGDRVTITCRASQDIRNDLGWYQQRPGKAPKFLIYSTSSLQSGVPSRFSGSGSGTDFILTISSLQPEDFATYYCLQSHNYPWTFGHGTKVEIK

SEQ ID NO: 230 - protein, 123 aa, Artificial Sequence
  synthetic construct; antigen binding domain
QVQLVESGGGVVQPGRSLRLSCAVSGFTLSSYGMDWVRQAPGKGLEWVAVIWYDGSNKYYSDSVKGRFTISRDNSKNTLFLQMNSLRADDTAVYYCARDGELGLDYYSGMDVWGQGTTVTVSS

SEQ ID NO: 231 - protein, 107 aa, Artificial Sequence
  synthetic construct; antigen binding domain
DIQMTQSPSSLSASVGDRVTITCRASQDIRNDLGWYQQKPGKAPKRLIYGASSLQSGVPSRFSGSGSGTEFTLTISSLQPEDFATYYCLQLNSYPRTFGQGTKVEIK

SEQ ID NO: 232 - protein, 118 aa, Artificial Sequence
  synthetic construct; antigen binding domain
QVQLVESGGGVVQPGRSLRLSCAASGFTFSSFGMHWVRQAPGKGLEWVAVISYDGRNRYYADSVKGRFTISRDNSKNTLYLQMNSLSAEDTAMFYCAKDGFGNSFDYWGQGTLVTVSS

SEQ ID NO: 233 - protein, 112 aa, Artificial Sequence
  synthetic construct; antigen binding domain
DVVMTQSPLSLPVTLGQPASISCRSSQSLLYSDGNTYLTWFQQRPGQSPRRLIYKVSNRDSGVPDRFSGSGSGTDFTLTISRVEAEDVGIYYCMQGTHWPWTFGQGTKVEIK

SEQ ID NO: 234 - protein, 123 aa, Artificial Sequence
  synthetic construct; antigen binding domain
QVQLVESGGGVVQPGRSLRLSCEASGFTFSSYGMHWVRQAPGKGLEWVAVIWYSESNKYYTDSMKGRLTISRDNSKNTLYLQMNSLRAEDTAVYYCARGGLLGKYYYYGMDVWGQGTTVTVSS

SEQ ID NO: 235 - protein, 107 aa, Artificial Sequence
  synthetic construct; antigen binding domain
DIQMTQSPSSLSASVGDRVIITCRASQDIRNDLGWYQQKPGKAPKRLIYAASSLQSGVPSRFSGSGSGTEFTLTISSLQPEDFATFYCLQLNSYPYTFGQGTKLEIK

SEQ ID NO: 236 - protein, 123 aa, Artificial Sequence
  synthetic construct; antigen binding domain
QVQLVESGGGVAQPGRSLSLSCAASGFTFSDYGMHWVRQAPGKGLEWVAVIWYAGSNKYYADSVKDRFTISRDNSKNTLYLQMRSLRVEDTAVYYCARGGELRLDYYSGLDVWGQGTTVTVSS

SEQ ID NO: 237 - protein, 107 aa, Artificial Sequence
  synthetic construct; antigen binding domain
DIQMTQSPSSLSASVGDRVTVTCRASQGIRSDLGWYQQKPGKAPKRLIYAASSFQSGVPSRFSGSGSGTEFTLTISSLHPEDFATYYCLQSNNYPWTFGQGTKVEIK

SEQ ID NO: 238 - protein, 124 aa, Artificial Sequence
  synthetic construct; antigen binding domain
QVQLVESGGGVVQPGGSLRLSCAVSGFTFSDYGMHWVRQVPGAGLEWVAVIYYEGSNKYYADSVKGRFTISRDNSKNTLYLQMNSLRVEDTSMYFCARGPLLGGNFYSYLMDVWGQGTTVTVSS

SEQ ID NO: 239 - protein, 107 aa, Artificial Sequence
  synthetic construct; antigen binding domain
AIQMTQSPSSLSASVGDRVTITCRASQGIRNGLGWYQQKPGKAPKLLIYTASSLQSGVPSRFSGSGSGTDFTLTISSLQPEDFATYYCLQDYNYPFSFGPGTKVDIK

SEQ ID NO: 240 - protein, 124 aa, Artificial Sequence
  synthetic construct; antigen binding domain
QVQLVESGGGVVQPGRSLRLSCAASGFTVRNYGMHWVRQAPGKGLEWVAVIWYDGSNKYYADSVKGRFTISRDNSKNTLFLQMNSLRAEDTAVYYCARGGELVRGDYYYGMDVWGQGTTVTVSS

SEQ ID NO: 241 - protein, 107 aa, Artificial Sequence
  synthetic construct; antigen binding domain
DIQMTQSPSSLSASVGDRVTITCRASQGIRNDLGWYQQKPGKAPKRLIYGASSLQSGVPSRFSGSGSGTEFTLTISSLQPEDFATYYCLQHNSYPYTFGQGTKLEIK

SEQ ID NO: 242 - protein, 117 aa, Artificial Sequence
  synthetic construct; antigen binding domain
QVQLVESGGGVVQPGRSLRLSCAASGTIFSTHGMHWVRQAPGKGLEWVAVISYDGNKKYYAGSVKGRFTISRDNSKNTLYLQMNDVRSEDTAVYHCTTDITGITDYWGQGTLVTVSS

SEQ ID NO: 243 - protein, 106 aa, Artificial Sequence
  synthetic construct; antigen binding domain
DIQMTQSPSSLSASVGDRVTITCRASQGIGNDLGWYQQKLGKAPKRLIYAASSLESGVPSRFSGSGSGTEFILTISSLQAEDFATYYCLQHNGFPTFGQGTKVEIK

SEQ ID NO: 244 - protein, 121 aa, Artificial Sequence
  synthetic construct; antigen binding domain
QVQLVESGGGVVQPGRSLRLSCAASGFTFSNYGIHWVRQPPGQGLEWVAVIWYAGSNKFYADSVKGRFTISRDNSKNSAYLQMNSLRAEDTAVYYCARAPLGYYYYGMDVWGQGTTVTVSS

SEQ ID NO: 245 - protein, 107 aa, Artificial Sequence
  synthetic construct; antigen binding domain
DIQMTQSPSSLSASVGDRVTITCRASQGIRNDLGWYQQKPGKAPKRLIYDASSLESGVPSRFSGSGSGTEFTLTISSLQPEDFATYYCLQHNSYPWTFGQGTKVEIK

SEQ ID NO: 246 - protein, 125 aa, Artificial Sequence
  synthetic construct; antigen binding domain
QVQLVESGGGVVQPGRSLRLSCAASGLTVSSYVMHWVRQAPGKGLEWVAIIWYDGSNKYYGDSVKGRFTISRDNSKKTLYLQMNSLRAEDTAVYYCARGRPLSSSSSDYYGLDVWGQGTTVTVSS

SEQ ID NO: 247 - protein, 107 aa, Artificial Sequence
  synthetic construct; antigen binding domain
AIQMTQSPSSLSASVGDRVTIICRASQGIRNDLGWYQQKPGKAPNLLIYAASSLQSGVPSRFSGSGSGTDFTLTISSLQPEDFATYYCLQDYNYPWTFGQGTKVEIK

SEQ ID NO: 248 - protein, 120 aa, Artificial Sequence
  synthetic construct; antigen binding domain
EVQLVESGGGLVQPGGSLRLSCAASGFTFSNYEMYWVRQAPGKGLEWVSYISSSGTTIYYADSVKGRFSVSRENARSSLYLQMNSLRVEDSAVYFCAKYNWNSFYGLDVWGQGTTVTVSS

SEQ ID NO: 249 - protein, 107 aa, Artificial Sequence
  synthetic construct; antigen binding domain
AIQMTQSPSSLSASVGDRVTITCRASQDIRNDLGWYQQKPGKAPKLLISAASSLQGGVPSRFSGSGSGTDFTLTISSLQPADFATYYCLQEYNYALTFGGGTKVEIK

SEQ ID NO: 250 - protein, 123 aa, Artificial Sequence
  synthetic construct; antigen binding domain
EVQLVESGGGLVQPGGSLRLSCAASGFTFRVYEMNWVRQAPGKGLEWISYIGSSGFTIYYADSVKGRFTISRDNAKNSLFLQLNSLRAEDTAVYYCARGWNDGVPNYLGMDVWGQGTTVTVSS

SEQ ID NO: 251 - protein, 107 aa, Artificial Sequence
  synthetic construct; antigen binding domain
DIQMTQSPSSLSASVGDRVTITCQASQDINKYLNWYQQKPGKAPKLLIYDASNLETGVPSRFSGSGSGTDFTFTISSLQPEDIARYHCQQYDKIPLTFGGGTKVEIK

SEQ ID NO: 252 - protein, 123 aa, Artificial Sequence
  synthetic construct; antigen binding domain
QVQLVESGGGVVQPGRSLRLSCAASGFTFSSYGMHWVRQAPGKGLEWVAVIWYVGSNKYYGESVKGRFTISRDNSKNTLYLQMNSLRDEDTAIYYCARGGQLGSFYYYGMDVWGQGTTVTVSS

SEQ ID NO: 253 - protein, 107 aa, Artificial Sequence
  synthetic construct; antigen binding domain
DIQMTQSPSSLSASVGDRVTITCRASQGIRNDLGWYQQKPGKAPKRLIYDVSSLQSGVPSRFSGSGSGTEFTLTISSLQPEDLATYYCLQHNSYPWTFGQGTKVEIK

SEQ ID NO: 254 - protein, 120 aa, Artificial Sequence
  synthetic construct; antigen binding domain
QVQLVESGGGVVQPGRSLRISCAASGFTFNNYGFHWVRQAPGRGLEWVAVIWYSGSNKYYGDSVKGRFTISRDNSKNILYLQMNSLRAEDTAIYYCARFPFSSSWLLDYWGQGTLVTVSS

SEQ ID NO: 255 - protein, 107 aa, Artificial Sequence
  synthetic construct; antigen binding domain
DIQLTQSPSFLSASVGDRVTFTCWASQGISDYLAWYQQKPGKAPKLLIYAASALQSGVPSRFSGSGSGTEFTLTVSSLQPEDFATYYCQQLNSYPFTFGPGTKVDIK

SEQ ID NO: 256 - protein, 119 aa, Artificial Sequence
  synthetic construct; antigen binding domain
QLQLQESGPGLVKPSETLSLTCTVSGGSISSTNHYWGWIRQPPGKGLEWIGNVYYIGNAYYNPSLKTGVTFSVDTSKNQFSLNLRSVTAADTAMYYCARLSNWNFLDLWGQGTLVTVSS

SEQ ID NO: 257 - protein, 106 aa, Artificial Sequence
  synthetic construct; antigen binding domain
EIVMTQSPATLSVSPGERATLSCRASQSISSNLAWYQQKPGQAPRLLIYGASTRATGIPARFSGSGSGTEFTLTISSLQSEDFAVYYCQQFNNWLSFGGGTKVEIK

SEQ ID NO: 258 - protein, 122 aa, Artificial Sequence
  synthetic construct; antigen binding domain
QVQLVESGGGVVQPGRSLRLSCAASGFTFSTYGMHWVRQAPGKGLEWVAVIWYVGSNKFYADSVKGRFTISRDNSKNTLYLQMDSLRAEDTGVYHCARDSMVRPYYYGMDVWGQGTTVTVSS

SEQ ID NO: 259 - protein, 108 aa, Artificial Sequence; identical to SEQ ID NO: 12
  synthetic construct; antigen binding domain

SEQ ID NO: 260 - protein, 125 aa, Artificial Sequence
  synthetic construct; antigen binding domain
QVQLVESGGGVVQPGRSLRLSCSASGFTLSNFVMHWVRQAPGKGLEWVAVILYDGSNKYYADSVKGRFTISRDNSNNRLYLQMNSLRAEDTALYYCARGESLGSPIYYYYGLDVWGQGTTVTVSS

SEQ ID NO: 261 - protein, 120 aa, Artificial Sequence
  synthetic construct; antigen binding domain
QVQLQESGPGLVKPSETLSLTCIVSGGSISGYFWNWIRQPPGKGLEWIGYIYYSGTTIYNPSLKSRFTISLDTSKNQFSLKLTSVTAADTAVYYCARESYNPSPRYFDHWGQGTLVTVSS

SEQ ID NO: 262 - protein, 125 aa, Artificial Sequence
  synthetic construct; antigen binding domain
QVQLVESGGGVVQPGRSLRLSCAASGFSFSSYGMHWVRQAPGKGLEWMAVIWYAGSNKFYADSVKGRFTISRDNSKNTLYLQMNSLTAEDTAVYYCARGSSLAAPDLYKYGMDVWGQGTTVTVSS

SEQ ID NO: 263 - protein, 117 aa, Artificial Sequence
  synthetic construct; antigen binding domain
QVQLQESGPGLVKPSETLSLTCTISGGSISNSFLTWIRQPPGKGLEWIGYIYHRGNTDSNPSLKSRVTISTDPSKNQFSLTLHSVTAADSAIYYCARGQFMEWFDFWGQGTLVTVSS

SEQ ID NO: 264 - protein, 125 aa, Artificial Sequence
  synthetic construct; antigen binding domain
QVQLVESGGGVVQPGRSLRVSCEASGFTLSSYGMNWVRQAPGKGLEWVAVIWYDGSNKYYSDSVKGRFTISRDNSKNTLYLQMNGLRDDDTAVYYCARGEQLGSHVYYYYGMDVWGQGTTVTVSS

SEQ ID NO: 265 - protein, 125 aa, Artificial Sequence
  synthetic construct; antigen binding domain
QVQLVESGGGVVQPGKSLRLSCAASGFTFSNYVMHWVRQTPGKGLEWVAIILFPGSNKYYVDSVQGRFTISRDNSKNTLSLQMNSLRAEDTAVYYCARGSSLTALDYYYYGLDVWGQGTTVTVSS

SEQ ID NO: 266 - protein, 125 aa, Artificial Sequence
  synthetic construct; antigen binding domain
QVQLVESGGGVVQPGRSLRLSCAASGFTFSNYVMHWVRQAPGKGLEWVAIIWYDGTNEDYADSVKVRFTISRDISKNTLYLQMNSLRAEDTAVYYCARDWFDCSSTSCYRYFDLWGRGTLVTVSS

SEQ ID NO: 267 - protein, 109 aa, Artificial Sequence
  synthetic construct; antigen binding domain
SLRLSCAASGFTFSNNNMHWVRQAPGKGLEWVAVIWYDGSNKDYVDSVKGRFTISRDNSKNTLYLQMNSLRAEDTAVYYCARFVVAPATYSYYYIIDVWGQGTTVTVSS

SEQ ID NO: 268 - protein, 126 aa, Artificial Sequence
  synthetic construct; antigen binding domain
QVQLVESGGGVVQPGRSLRLSCAASGFTFSTYGMHWVRQAPGKGLEWVAVISYDGRIKYYEDSVKGRFIISRDNSKNTLYLQVNTLRAEDTAVYYCAKERRYCSDTNTCSDVFDVWGQGTMVTVSS

SEQ ID NO: 269 - protein, 11 aa, Mus musculus
CASSRNTEVFF

SEQ ID NO: 270 - protein, 12 aa, Mus musculus
CASSIGNTEVFF

SEQ ID NO: 271 - protein, 14 aa, Mus musculus
CASSQPGKNTEVFF

SEQ ID NO: 272 - protein, 15 aa, Mus musculus
CASSLGQGNNSPLYF

SEQ ID NO: 273 - protein, 15 aa, Mus musculus
CASSQGQGGAETLYF

SEQ ID NO: 274 - protein, 13 aa, Mus musculus
CASSPPMGGQLYF

SEQ ID NO: 275 - protein, 14 aa, Mus musculus
CASSQEGANTEVFF

SEQ ID NO: 276 - protein, 15 aa, Mus musculus
CASSQVQGTGNTLYF

SEQ ID NO: 277 - protein, 14 aa, Mus musculus
CASSQEGDGYEQYF

SEQ ID NO: 278 - protein, 13 aa, Mus musculus
CTSAEGGGTEVFF

SEQ ID NO: 279 - protein, 14 aa, Mus musculus
CASSPPGGGTEVGG

SEQ ID NO: 280 - protein, 14 aa, Mus musculus
CASSGTDNQDTQYF

SEQ ID NO: 281 - protein, 14 aa, Mus musculus
CASSPGTGGYEQYF

SEQ ID NO: 282 - protein, 14 aa, Mus musculus
CASSLELGFYEQYF

SEQ ID NO: 283 - protein, 15 aa, Mus musculus
CASSLGGAPNERLFF

SEQ ID NO: 284 - protein, 14 aa, Mus musculus
CASSQEGDSYEQYF

SEQ ID NO: 285 - protein, 11 aa, Mus musculus
CASSRNTEVFF

SEQ ID NO: 286 - protein, 16 aa, Mus musculus
CASGDAMGGRDYAEQF

SEQ ID NO: 287 - protein, 12 aa, Mus musculus
CGAREGQDTQYF

SEQ ID NO: 288 - protein, 11 aa, Mus musculus
CGARTGGEQYF

SEQ ID NO: 289 - protein, 12 aa, Mus musculus
CTCSAGNQAPLF

SEQ ID NO: 290 - protein, 14 aa, Mus musculus
CASSGTGGGAEQFF

SEQ ID NO: 291 - protein, 15 aa, Mus musculus
CASSDEGGGTGQLYF

SEQ ID NO: 292 - protein, 16 aa, Mus musculus
CASSRDWGGSQNTLYF

SEQ ID NO: 293 - protein, 14 aa, Mus musculus
CASSPTGYNSPLYF

SEQ ID NO: 294 - protein, 15 aa, Mus musculus
CASSQVQGSAETLYF

SEQ ID NO: 295 - protein, 15 aa, Mus musculus
CASSGTGGNQDTQYF

SEQ ID NO: 296 - protein, 16 aa, Mus musculus
CASGDAGTGNYAEQFF

SEQ ID NO: 297 - protein, 15 aa, Mus musculus
CASSLRTGYNSPLYF

SEQ ID NO: 298 - protein, 14 aa, Mus musculus
CASRLGGDQNTLYF

SEQ ID NO: 299 - protein, 12 aa, Mus musculus
CASKTGGYEQYF

SEQ ID NO: 300 - protein, 11 aa, Mus musculus
CASSEGDTLYF

SEQ ID NO: 301 - protein, 15 aa, Mus musculus
CASSPGTFNQDTQYF

SEQ ID NO: 302 - protein, 13 aa, Mus musculus
CASASWTGDEQYF

SEQ ID NO: 303 - protein, 14 aa, Mus musculus
CASSLPGSQNTLYF

SEQ ID NO: 304 - protein, 14 aa, Mus musculus
CASSRDWAQDTQYF

SEQ ID NO: 305 - protein, 14 aa, Mus musculus
CASSDNWGAGEQYF

SEQ ID NO: 306 - protein, 14 aa, Mus musculus
CASSSGTASDTQYF

SEQ ID NO: 307 - protein, 15 aa, Mus musculus
CASSQTRDWGYEQYF

SEQ ID NO: 308 - protein, 14 aa, Mus musculus
CTCSGGLGGLEQYF

SEQ ID NO: 309 - protein, 14 aa, Mus musculus
CASSLGTGGIEQYF

SEQ ID NO: 310 - protein, 15 aa, Mus musculus
CASSLSDSNQDTQYF

SEQ ID NO: 311 - protein, 14 aa, Mus musculus
CASSERGGRDTQYF

SEQ ID NO: 312 - protein, 15 aa, Mus musculus
CTCSAVREGNSPLYF

SEQ ID NO: 313 - protein, 15 aa, Mus musculus
CASSLTGVSNERLFF

SEQ ID NO: 314 - protein, 13 aa, Mus musculus
CASSRQLNSDYTF

SEQ ID NO: 315 - protein, 15 aa, Mus musculus
CASSLRQGSNTEVFF

SEQ ID NO: 316 - protein, 16 aa, Mus musculus
CASSQNRDISAETLYF

SEQ ID NO: 317 - protein, 13 aa, Mus musculus
CASSWTANTEVFF

SEQ ID NO: 318 - protein, 15 aa, Mus musculus
CASSLRDWGQDTQYF

SEQ ID NO: 319 - protein, 15 aa, Mus musculus
CASSHWGGTTGQLYF

SEQ ID NO: 320 - protein, 15 aa, Mus musculus
CASSYSKGSAETLYF

SEQ ID NO: 321 - protein, 13 aa, Mus musculus
CAVSMINYNVLYF

SEQ ID NO: 322 - protein, 12 aa, Mus musculus
CASSDGQNTLYF

SEQ ID NO: 323 - protein, 13 aa, Mus musculus
CASSQEGPGQLYF

SEQ ID NO: 324 - protein, 14 aa, Mus musculus
CASTGQGYNSPLYF